European Patent Specification EP 3 310 368 B1, published July 16, 2025. Title: SINDBIS CONTROL VIRUS. Applicant: SERACARE LIFE SCIENCES, INC. The sequence listing filed with the application follows.

SEQUENCE LISTING (16 sequences)

SEQ ID NO: 1 - DNA, 10052 bp, Artificial Sequence
  Description of Artificial Sequence: Synthetic polynucleotide
attgacggcgtagtacacactattgaatcaaacagccgaccaattgcactaccatcacaatggagaagccagtagtaaacgtagacgtagacccccagagtccgtttgtcgtgcaactgcaaaaaagcttcccgcaatttgaggtagtagcacagcaggtcactccaaatgaccatgctaatgccagagcattttcgcatctggccagtaaactaatcgagctggaggttcctaccacagcgacgatcttggacataggcagcgcaccggctcgtagaatgttttccgagcaccagtatcattgtgtctgccccatgcgtagtccagaagacccggaccgcatgatgaaatacgccagtaaactggcggaaaaagcgtgcaagattacaaacaagaacttgcatgagaagattaaggatctccggaccgtacttgatacgccggatgctgaaacaccatcgctctgctttcacaacgatgttacctgcaacatgcgtgccgaatattccgtcatgcaggacgtgtatatcaacgctcccggaactatctatcatcaggctatgaaaggcgtgcggaccctgtactggattggcttcgacaccacccagttcatgttctcggctatggcaggttcgtaccctgcgtacaacaccaactgggccgacgagaaagtccttgaagcgcgtaacatcggactttgcagcacaaagctgagtgaaggtaggacaggaaaattgtcgataatgaggaagaaggagttgaagcccgggtcgcgggtttatttctccgtaggatcgacactttatccagaacacagagccagcttgcagagctggcatcttccatcggtgttccacttgaatggaaagcagtcgtacacttgccgctgtgatacagtggtgagttgcgaaggctacgtagtgaagaaaatcaccatcagtcccgggatcacgggagaaaccgtgggatacgcggttacacacaatagcgagggcttcttgctatgcaaagttactgacacagtaaaaggagaacgggtatcgttccctgtgtgcacgtacatcccggccaccatatgcgatcagatgactggtataatggccacggatatatcacctgacgatgcacaaaaacttctggttgggctcaaccagcgaattgtcattaacggtaggactaacaggaacaccaacaccatgcaaaattaccttctgccgatcatagcacaagggttcagcaaatgggctaaggagcgcaaggatgatcttgataacgagaaaatgctgggtactagagaacgcaagcttacgtatggctgcttgtgggcgtttcgcactaagaaagtacattcgttttatcgcccacctggaacgcagacctgcgtaaaagtcccagcctcttttagcgcttttcccatgtcgtccgtatggacgacctctttgcccatgtcgctgaggcagaaattgaaactggcattgcaaccaaagaaggaggaaaaactgctgcaggtctcggaggaattagtcatggaggccaaggctgcttttgaggatgctcaggaggaagccagagcggagaagctccgagaagcacttccaccattagtggcagacaaaggcatcgaggcagccgcagaagttgtctgcgaagtggaggggctccaggcggacatcggagcagcattagttgaaaccccgcgcggtcacgtaaggataatacctcaagcaaatgaccgtatgatcggacagtatatcgttgtctcgccaaactctgtgctgaagaatgccaaactcgcaccagcgcacccgctagcagatcaggttaagatcataacacactccggaagatcaggaaggtacgcggtcgaaccatacgacgctaaagtactgatgccagcaggaggtgccgtaccatggccagaattcctagcactgagtgagagcgccacgttagtgtacaacgaaagagagtttgtgaaccgcaaactataccacattgccatgcatggccccgccaagaatacagaagaggagcagtacaaggttacaaaggcagagcttgcagaaacagagtacgtgtttgacgtggacaagaagcgttgcgttaagaaggaagaagcctcaggtctggtcctctcgggagaactgaccaaccctccctatcatgagctagctctggagggactgaagacccgacctgcggtcccgtacaaggtcgaaacaataggagtgataggcacaccggggtcgggcaagtcagctattatcaagtcaactgtcacggcacgagatcttgttaccagcggaaagaaagaaaattgtcgcgaaattgaggccgacgtgctaagactgaggggtatgcagattacgtcgaagacagtagattcggttatgctcaacggatgccacaaagccgtagaagtgctgtacgttgacgaagcgttcgcgtgccacgcaggagcactacttgccttgattgctatcgtcaggccccgcaagaaggtagtactatgcggagaccccatgcaatgcggattcttcaacatgatgcaactaaaggtacatttcaatcaccctgaaaaagacatatgcaccaagacattctacaagtatatctcccggcgttgcacacagccagttacagctattgtatcgacactgcattacgatggaaagatgaaaaccacgaacccgtgcaagaagaacattgaaatcgatattacaggggccacaaagccgaagccaggggatatcatcctgacatgtttccgcgggtgggttaagcaattgcaaatcgactatcccggacatgaagtaatgacagccgcggcctcacaagggctaaccagaaaaggagtgtatgccgtccggcaaaaagtcaatgaaaacccactgtacgcgatcacatcagagcatgtgaacgtgttgctcacccgcactgaggacaggctagtgtggaaaaccttgcagggcgacccatggattaagcagcccactaacatacctaaaggaaactttcaggctactatagaggactgggaagctgaacacaagggaataattgctgcaataaacagccccactccccgtgccaatccgttcagctgcaagaccaacgtttgctgggcgaaagcattggaaccgatactagccacggccggtatcgtacttaccggttgccagtggagcgaactgttcccacagtttgcggatgacaaaccacattcggccatttacgccttagacgtaatttgcattaagtttttcggcatggacttgacaagcggactgttttctaaacagagcatcccactaacgtaccatcccgccgattcagcgaggccggtagctcattgggacaacagcccaggaacccgcaagtatgggtacgatcacgccattgccgccgaactctcccgtagatttccggtgttccagctagctgggaagggcacacaacttgatttgcagacggggagaaccagagttatctctgcacagcataacctggtcccggtgaaccgcaatcttcctcacgccttagtccccgagtacaaggagaagcaacccggcccggtcaaaaaattcttgaaccagttcaaacaccactcagtacttgtggtatcagaggaaaaaattgaagctccccgtaagagaatcgaatggatcgccccgattggcatagccggtgcagataagaactacaacctggctttcgggtttccgccgcaggcacggtacgacctggtgttcatcaacattggaactaaatacagaaaccaccactttcagcagtgcgaagaccatgcggcgaccttaaaaaccctttcgcgttcggccctgaattgccttaacccaggaggcaccctcgtggtgaagtcctatggctacgccgaccgcaacagtgaggacgtagtcaccgctcttgccagaaagtttgtcagggtgtctgcagcgagaccagattgtgtctcaagcaatacagaaatgtacctgattttccgacaactagacaacagccgtacacggcaattcaccccgcaccatctgaattgcgtgatttcgtccgtgtatgagggtacaagagatggagttggagccgcgccgtcataccgcaccaaaagggagaatattgctgactgtcaagaggaagcagttgtcaacgcagccaatccgctgggtagaccaggcgaaggagtctgccgtgccatctataaacgttggccgaccagttttaccgattcagccacggagacaggcaccgcaagaatgactgtgtgcctaggaaagaaagtgatccacgcggtcggccctgatttccggaagcacccagaagcagaagccttgaaattgctacaaaacgcctaccatgcagtggcagacttagtaaatgaacataacatcaagtctgtcgccattccactgctatctacaggcatttacgcagccggaaaagaccgccttgaagtatcacttaactgcttgacaaccgcgctagacagaactgacgcggacgtaaccatctattgcctggataagaagtggaaggaaagaatcgacgcggcactccaacttaaggagtctgtaacagagctgaaggatgaagatatggagatcgacgatgagttagtatggattcatccagacagttgcttgaagggaagaaagggattcagtactacaaaaggaaaattgtattcgtacttcgaaggcaccaaattccatcaagcagcaaaagacatggcggagataaaggtcctgttccctaatgaccaggaaagtaatgaacaactgtgtgcctacatattgggtgagaccatggaagcaatccgcgaaaagtgcccggtcgaccataacccgtcgtctagcccgcccaaaacgttgccgtgcctttgcatgtatgccatgacgccagaaagggtccacagacttagaagcaataacgtcaaagaagttacagtatgctcctccaccccccttcctaagcacaaaattaagaatgttcagaaggttcagtgcacgaaagtagtcctgtttaatccgcacactcccgcattcgttcccgcccgtaagtacatagaagtgccagaacagcctaccgctcctcctgcacaggccgaggaggcccccgaagttgtagcgacaccgtcaccatctacagctgataacacctcgcttgatgtcacagacatctcactggatatggatgacagtagcgaaggctcacttttttcgagctttagcggatcggacaactctattactagtatggacagttggtcgtcaggacctagttcactagagatagtagaccgaaggcaggtggtggtggctgacgttcatgccgtccaagagcctgcccctattccaccgccaaggctaaagaagatggcccgcctggcagcggcaagaaaagagcccactccaccggcaagcaatagctctgagtccctccacctctcttttggtggggtatccatgtccctcggatcaattttcgacggagagacggcccgccaggcagcggtacaacccctggcaacaggccccacggatgtgcctatgtctttcggatcgttttccgacggagagattgatgagctgagccgcagagtaactgagtccgaacccgtcctgtttggatcatttgaaccgggcgaagtgaactcaattatatcgtcccgatcagccgtatcttttccactacgcaagcagagacgtagacgcaggagcaggaggactgaatactgactaaccggggtaggtgggtacatattttcgacggacacaggccctgggcacttgcaaaagaagtccgttctgcagaaccagcttacagaaccgaccttggagcgcaatgtcctggaaagaattcatgccccggtgctcgacacgtcgaaagaggaacaactcaaactcaggtaccagatgatgcccaccgaagccaacaaaagtaggtaccagtctcgtaaagtagaaaatcagaaagccataaccactgagcgactactgtcaggactacgactgtataactctgccacagatcagccagaatgctataagatcacctatccgaaaccattgtactccagtagcgtaccggcgaactactccgatccacagttcgctgtagctgtctgtaacaactatctgcatgagaactatccgacagtagcatcttatcagattactgacgagtacgatgcttacttggatatggtagacgggacagtcgcctgcctggatactgcaaccttctgccccgctaagcttagaagttacccgaaaaaacatgagtatagagccccgaatatccgcagtgcggttccatcagcgatgcagaacacgctacaaaatgtgctcattgccgcaactaaaagaaattgcaacgtcacgcagatgcgtgaactgccaacactggactcagcgacattcaatgtcgaatgctttcgaaaatatgcatgtaatgacgagtattgggaggagttcgctcggaagccaattaggattaccactgagtttgtcaccgcatatgtagctagactgaaaggccctaaggccgccgcactatttgcaaagacgtataatttggtcccattgcaagaagtgcctatggatagattcgtcatggacatgaaaagagacgtgaaagttacaccaggcacgaaacacacagaagaaagaccgaaagtacaagtgatacaagccgcagaacccctggcgactgcttacttatgcgggattcaccgggaattagtgcgtaggcttacggccgtcttgcttccaaacattcacacgctttttgacatgtcggcggaggattttgatgcaatcatagcagaacacttcaagcaaggcgacccggtactggagacggatatcgcatcattcgacaaaagccaagacgacgctatggcgttaaccggtctgatgatcttggaggacctgggtgtggatcaaccactactcgacttgatcgagtgcgcctttggagaaatatcatccacccatctacctacgggtactcgttttaaattcggggcgatgatgaaatccggaatgttcctcacactttttgtcaacacagttttgaatgtcgttatcgccagcagagtactagaagagcggcttaaaacgtccagatgtgcagcgttcattggcgacgacaacatcatacatggagtagtatctgacaaagaaatggctgagaggtgcgccacctggctcaacatggaggttaagatcatcgacgcagtcatcggtgagagaccaccttacttctgcggcggatttatcttgcaagattcggttacttccacagcgtgccgcgtggcggatcccctgaaaaggctgtttaagttgggtaaaccgctcccagccgacgacgagcaagacgaagacagaagacgcgctctgctagatgaaacaaaggcgtggtttagagtaggtataacaggcactttagcagtggccgtgacgacccggtatgaggtagacaatattacacctgtcctactggcattgagaacttttgcccagagcaaaagagcattccaagccatcagaggggaaataaagcatctctacggtggtcctaaatagtcagcatagtacatttcatctgactaatactacaacaccaccacctctagagtttaaacaggcctggcgcgccacgtgacgcgtgcatgcatttaaatatcgagggcaggagcgagagggccaaggccagggagggcggccaccaccatcaccaccatcaccattagtaatgaggtaaccgtggggcccaatgatccgaccagcaaaactcgatgtacttccgaggaactgatgtgcataatgcatcaggctggtacattagatccccgcttaccgcgggcaatatagcaacactaaaaactcgatgtacttccgaggaagcgcagtgcataatgctgcgcagtgttgccacataaccactatattaaccatttatctagcggacgccaaaaactcaatgtatttctgaggaagcgtggtgcataatgccacgcagcgtctgcataacttttattatttcttttattaatcaacaaaattttgtttttaacatttcaaaaaaaaaaaaaaaaaaaaaaaaaaaaaaaaaaaaagggaattcctcgattaattaagcggccgctcgaggggaattaattcttgaagacgaaagggccaggtggcacttttcggggaaatgtgcgcggaacccctatttgtttatttttctaaatacattcaaatatgtatccgctcatgagacaataaccctgataaatgcttcaataatattgaaaaaggaagagtatgagtattcaacatttccgtgtcgcccttattcccttttttgcggcattttgccttcctgtttttgctcacccagaaacgctggtgaaagtaaaagatgctgaagatcagttgggtgcacgagtgggttacatcgaactggatctcaacagcggtaagatccttgagagttttcgccccgaagaacgttttccaatgatgagcacttttaaagttctgctatgtggcgcggtattatcccgtgttgacgccgggcaagagcaactcggtcgccgcatacactattctcagaatgacttggttgagtactcaccagtcacagaaaagcatcttacggatggcatgacagtaagagaattatgcagtgctgccataaccatgagtgataacactgcggccaacttacttctgacaacgatcggaggaccgaaggagctaaccgcttttttgcacaacatgggggatcatgtaactcgccttgatcgttgggaaccggagctgaatgaagccataccaaacgacgagcgtgacaccacgatgcctgtagcaatggcaacaacgttgcgcaaactattaactggcgaactacttactctagcttcccggcaacaattaatagactggatggaggcggataaagttgcaggaccacttctgcgctcggcccttccggctggctggtttattgctgataaatctggagccggtgagcgtgggtctcgcggtatcattgcagcactggggccagatggtaagccctcccgtatcgtagttatctacacgacggggagtcaggcaactatggatgaacgaaatagacagatcgctgagataggtgcctcactgattaagcattggtaactgtcagaccaagtttactcatatatactttagattgatttaaaacttcatttttaatttaaaaggatctaggtgaagatcctttttgataatctcatgaccaaaatcccttaacgtgagttttcgttccactgagcgtcagaccccgtagaaaagatcaaaggatcttcttgagatcctttttttctgcgcgtaatctgctgcttgcaaacaaaaaaaccaccgctaccagcggtggtttgtttgccggatcaagagctaccaactctttttccgaaggtaactggcttcagcagagcgcagataccaaatactgtccttctagtgtagccgtagttaggccaccacttcaagaactctgtagcaccgcctacatacctcgctctgctaatcctgttaccagtggctgctgccagtggcgataagtcgtgtcttaccgggttggactcaagacgatagttaccggataaggcgcagcggtcgggctgaacggggggttcgtgcacacagcccagcttggagcgaacgacctacaccgaactgagatacctacagcgtgagcattgagaaagcgccacgcttcccgaagggagaaaggcggacaggtatccggtaagcggcagggtcggaacaggagagcgcacgagggagcttccagggggaaacgcctggtatctttatagtcctgtcgggtttcgccacctctgacttgagcgtcgatttttgtgatgctcgtcaggggggcggagcctatggaaaaacgccagcaacgcgagctcgtatggacatattgtcgttagaacgcggctacaattaatacataaccttatgtatcatacacatacgatttaggggacactatag

SEQ ID NO: 2 - DNA, 1950 bp, Zaire ebolavirus
aggaatattgcagttacctcgtgatcgattcaagaggacatcattctttctttgggtaattatccttttccaaagaacattttccatcccgcttggagttatccacaatagtacattacaggttagtgatgtcgacaaactagtttgtcgtgacaaactgtcatccacaaatcaattgagatcagttggactgaatctcgaggggaatggagtggcaactgacgtgccatctgcgactaaaagatggggcttcaggtccggtgtcccaccaaaggtggtcaattatgaagctggtgaatgggctgaaaactgctacaatcttgaaatcaaaaaacctgacgggagtgagtgtctaccagcagcgccagacgggattcggggcttcccccggtgccggtatgtgcacaaagtatcaggaacgggaccatgtgccggagactttgccttccacaaagagggtgctttcttcctgtatgatcgacttgcttccacagttatctaccgaggaacgactttcgctgaaggtgtcgttgcatttctgatactgccccaagctaagaaggacttcttcagctcacaccccttgagagagccggtcaatgcaacggaggacccgtcgagtggctattattctaccacaattagatatcaggctaccggttttggaactaatgagacagagtacttgttcgaggttgacaatttgacctacgtccaacttgaatcaagattcacaccacagtttctgctccagctgaatgagacaatatatgcaagtgggaagaggagcaacaccacgggaaaactaatttggaaggtcaaccccgaaattgatacaacaatcggggagtgggccttcagggaaactaaaaaaacctcactagaaaaattcgcagtgaagagttgtctttcacagctgtatcaaacggacccaaaaacatcagtggtcagagtccggcgcgaacttcttccgacccagagaccaacacaacaaatgaagaccacaaaatcatggcttcagaaaattcctctgcaatggttcaagtgcacagtcaaggaaggaaagctgcagtgtcgcatctgacaacccttgccacaatctccacgagtcctcaacctcccacaaccaaaacaggtccggacaacagcacccataatacacccgtgtataaacttgacatctctgaggcaactcaagttggacaacatcaccgtagagcagacaacgacagcacagcctccgacactccccccgccacgaccgcagccggacccttaaaagcagagaacaccaacacgagtaagagcgctgactccctggacctcgccaccacgataagcccccaaaactacagcgagactgctggcaacaacaacactcatcaccaagataccggagaagagagtgccagcagcgggaagctaggcttaattaccaatactattgctggagtagcaggactgatcacaggcgggagaaggactcgaagagaagtaattgtcaatgctcaacccaaatgcaaccccaatttacattactggactactcaggatgaaggtgctgcaatcggattggcctggataccatatttcgggccagcagccgaaggaatttacacagaggggctaatgcacaaccaagatggtttaatctgtgggttgaggcagctggccaacgaaacgactcaagctctccaactgttcctgagagccacaactgagctgcgaaccttttcaatcctcaaccgtaaggcaattgacttcctgctgcagcgatggggtggcacatgccacattttgggaccggactgctgtatcgaaccacatgattggaccaagaacataacagacaaaattgatcagattattcatgattttgttgataaaacccttccggaccagggggacaatgacaattggtggacaggatggagacaatggataccggca

SEQ ID NO: 3 - DNA, 2217 bp, Artificial Sequence
  Description of Artificial Sequence: Synthetic polynucleotide
  MISC_FEATURE (1)..(1577): Ebola NP gene sequence
  MISC_FEATURE (1578)..(2127): Ebola VP24 sequence
  MISC_FEATURE (2128)..(2217): Human RNAse P internal control sequence
tactgtaatcatacctggtttgtttcagagccatatcaccaagatagagaacaacctaggtctccggagggggcaagggcatcagtgtgctcagttgaaaatcccttgtcaacatctaggccttatcacatcacaagttccgccttaaactctgcagggtgatccaacaaccttaatagcaacattattgttaaaggacagcattagttcacagtcaaacaagcaagattgagaattaactttgattttgaacctgaacacccagaggactggagactcaacaaccctaaagcctggggtaaaacattagaaatagtttaaagacaaattgctcggaatcacaaaattccgagtatggattctcgtcctcagaaagtctggtagacgccgagtctcactgaatctgacatggattaccacaagatcttgacagcaggtctgtccgttcaacaggggattgttcggcaaagagtcatcccagtgtatcaagtaaacaatcttgaggaaatttgccaacttatcatacaggcctttgaagctggtgttgattttcaagagagtgcggacagtttccttctcatgctttgtcttcatcatgcgtaccaaggagattacaaacttttcttggaaagtggcgcagtcaagtatttggaagggcacgggttccgttttgaagtcaagaagcgtgatggagtgaagcgccttgaggaattgctgccagcagtatctagtgggagaaacattaagagaacacttgctgccatgccggaagaggagacgacttaatgccggacatgatgccaacgatgctgtgatttcaaattcagtggctcaagctcgtttttcaggtctattgattgtcaaaacagtacttgatcatatcctacaaaagacagaacgaggagttcgtctccatcctcttgcaaggaccgccaaggtaaaaaatgaggtgaactccttcaaggctgcactcagctccctggccaagcatggagagtatgctcctttcgcccgacttttgaacctttctggagtaaataatcttgagcatggtcttttccctcaactgtcggcaattgcactcggagtcgccacagcccacgggagcaccctcgcaggagtaaatgttggagaacagtatcaacagctcagagaggcagccactgaggctgagaagcaactccaacaatatgcggagtctcgtgaacttgaccatcttggacttgatgatcaggaaaagaaaattcttatgaacttccatcagaaaaagaacgaaatcagcttccagcaaacaaacgcgatggtaactctaagaaaagagcgcctggccaagctgacagaagctatcactgctgcatcactgcccaaaacaagtggacattacgatgatgatgacgacattccctttccaggacccatcaatgatgacgacaatcctggccatcaagatgatgatccgactgactcacaggatacgaccattcccgatgtggtagttgatcccgatgatggaggctacggcgaataccaaagttactcggaaaacggcatgagtgcaccagatgacttggtcctatgtcttttagctgtataccagttgcccctgagatacgccacaaaagtgtctctgagctaaagtggtctgtacacatctcatacattgtattaggggcaataatatctaattgaacttagccatttaaaatttagtgcataaatctgggctaactccaccaggtcaactccattggctgaaaagaagcccacctacaacgaacattactttgagcgccctcacaattaaaaaataagagcgtcgttccaacaatcgagcgcaaggttacaaggttgaactgagagtgtctagacaacaaaatatcgatactccagacaccaagcaagacctgagaaaaaaccatggccaaagctacgggacgatacaatctaatatcgcccaaaaaggacctggagaaaggggttgtcttaagcgacctctgtaacttcttagttagtcaaactattcaagggtggaaagtttattgggctggtattgagtttgatgtgactcacaaaggaatggccctattgcatagactgaaaactaatgactttgcccctgcatggtcatggcggtgtttgcagatttggacctgcgagcgggttctgacctgaaggctctgcgcggacttgtggagacagccgctcaccttggctatt

SEQ ID NO: 4 - DNA, 9719 bp, Human immunodeficiency virus
tggaagggctaattcactcccaacgaagacaagatatccttgatctgtggatctaccacacacaaggctacttccctgattagcagaactacacaccagggccagggatcagatatccactgacctttggatggtgctacaagctagtaccagttgagccagagaagttagaagaagccaacaaaggagagaacaccagcttgttacaccctgtgagcctgcatggaatggatgacccggagagagaagtgttagagtggaggtttgacagccgcctagcatttcatcacatggcccgagagctgcatccggagtacttcaagaactgctgacatcgagcttgctacaagggactttccgctggggactttccagggaggcgtggcctgggcgggactggggagtggcgagccctcagatcctgcatataagcagctgctttttgcctgtactgggtctctctggttagaccagatctgagcctgggagctctctggctaactagggaacccactgcttaagcctcaataaagcttgccttgagtgcttcaagtagtgtgtgcccgtctgttgtgtgactctggtaactagagatccctcagacccttttagtcagtgtggaaaatctctagcagtggcgcccgaacagggacctgaaagcgaaagggaaaccagaggagctctctcgacgcaggactcggcttgctgaagcgcgcacggcaagaggcgaggggcggcgactggtgagtacgccaaaaattttgactagcggaggctagaaggagagagatgggtgcgagagcgtcagtattaagcgggggagaattagatcgatgggaaaaaattcggttaaggccagggggaaagaaaaaatataaattaaaacatatagtatgggcaagcagggagctagaacgattcgcagttaatcctggcctgttagaaacatcagaaggctgtagacaaatactgggacagctacaaccatcccttcagacaggatcagaagaacttagatcattatataatacagtagcaaccctctattgtgtgcatcaaaggatagagataaaagacaccaaggaagctttagacaagatagaggaagagcaaaacaaaagtaagaaaaaagcacagcaagcagcagctgacacaggacacagcaatcaggtcagccaaaattaccctatagtgcagaacatccaggggcaaatggtacatcaggccatatcacctagaactttaaatgcatgggtaaaagtagtagaagagaaggctttcagcccagaagtgatacccatgttttcagcattatcagaaggagccaccccacaagatttaaacaccatgctaaacacagtggggggacatcaagcagccatgcaaatgttaaaagagaccatcaatgaggaagctgcagaatgggatagagtgcatccagtgcatgcagggcctattgcaccaggccagatgagagaaccaaggggaagtgacatagcaggaactactagtacccttcaggaacaaataggatggatgacaaataatccacctatcccagtaggagaaatttataaaagatggataatcctgggattaaataaaatagtaagaatgtatagccctaccagcattctggacataagacaaggaccaaaggaaccctttagagactatgtagaccggttctataaaactctaagagccgagcaagcttcacaggaggtaaaaaattggatgacagaaaccttgttggtccaaaatgcgaacccagattgtaagactattttaaaagcattgggaccagcggctacactagaagaaatgatgacagcatgtcagggagtaggaggacccggccataaggcaagagttttggctgaagcaatgagccaagtaacaaattcagctaccataatgatgcagagaggcaattttaggaaccaaagaaagattgttaagtgtttcaattgtggcaaagaagggcacacagccagaaattgcagggcccctaggaaaaagggctgttggaaatgtggaaaggaaggacaccaaatgaaagattgtactgagagacaggctaattttttagggaagatctggccttcctacaagggaaggccagggaattttcttcagagcagaccagagccaacagccccaccagaagagagcttcaggtctggggtagagacaacaactccccctcagaagcaggagccgatagacaaggaactgtatcctttaacttccctcaggtcactctttggcaacgacccctcgtcacaataaagataggggggcaactaaaggaagctctattagatacaggagcagatgatacagtattagaagaaatgagtttgccaggaagatggaaaccaaaaatgatagggggaattggaggttttatcaaagtaagacagtatgatcagatactcatagaaatctgtggacataaagctataggtacagtattagtaggacctacacctgtcaacataattggaagaaatctgttgactcagattggttgcactttaaattttcccattagccctattgagactgtaccagtaaaattaaagccaggaatggatggcccaaaagttaaacaatggccattgacagaagaaaaaataaaagcattagtagaaatttgtacagagatggaaaaggaagggaaaatttcaaaaattgggcctgaaaatccatacaatactccagtatttgccataaagaaaaaagacagtactaaatggagaaaattagtagatttcagagaacttaataagagaactcaagacttctgggaagttcaattaggaataccacatcccgcagggttaaaaaagaaaaaatcagtaacagtactggatgtgggtgatgcatatttttcagttcccttagatgaagacttcaggaagtatactgcatttaccatacctagtataaacaatgagacaccagggattagatatcagtacaatgtgcttccacagggatggaaaggatcaccagcaatattccaaagtagcatgacaaaaatcttagagccttttagaaaacaaaatccagacatagttatctatcaatacatggatgatttgtatgtaggatctgacttagaaatagggcagcatagaacaaaaatagaggagctgagacaacatctgttgaggtggggacttaccacaccagacaaaaaacatcagaaagaacctccattcctttggatgggttatgaactccatcctgataaatggacagtacagcctatagtgctgccagaaaaagacagctggactgtcaatgacatacagaagttagtggggaaattgaattgggcaagtcagatttacccagggattaaagtaaggcaattatgtaaactccttagaggaaccaaagcactaacagaagtaataccactaacagaagaagcagagctagaactggcagaaaacagagagattctaaaagaaccagtacatggagtgtattatgacccatcaaaagacttaatagcagaaatacagaagcaggggcaaggccaatggacatatcaaatttatcaagagccatttaaaaatctgaaaacaggaaaatatgcaagaatgaggggtgcccacactaatgatgtaaaacaattaacagaggcagtgcaaaaaataaccacagaaagcatagtaatatggggaaagactcctaaatttaaactgcccatacaaaaggaaacatgggaaacatggtggacagagtattggcaagccacctggattcctgagtgggagtttgttaatacccctcccttagtgaaattatggtaccagttagagaaagaacccatagtaggagcagaaaccttctatgtagatggggcagctaacagggagactaaattaggaaaagcaggatatgttactaatagaggaagacaaaaagttgtcaccctaactgacacaacaaatcagaagactgagttacaagcaatttatctagctttgcaggattcgggattagaagtaaacatagtaacagactcacaatatgcattaggaatcattcaagcacaaccagatcaaagtgaatcagagttagtcaatcaaataatagagcagttaataaaaaaggaaaaggtctatctggcatgggtaccagcacacaaaggaattggaggaaatgaacaagtagataaattagtcagtgctggaatcaggaaagtactatttttagatggaatagataaggcccaagatgaacatgagaaatatcacagtaattggagagcaatggctagtgattttaacctgccacctgtagtagcaaaagaaatagtagccagctgtgataaatgtcagctaaaaggagaagccatgcatggacaagtagactgtagtccaggaatatggcaactagattgtacacatttagaaggaaaagttatcctggtagcagttcatgtagccagtggatatatagaagcagaagttattccagcagaaacagggcaggaaacagcatattttcttttaaaattagcaggaagatggccagtaaaaacaatacatactgacaatggcagcaatttcaccggtgctacggttagggccgcctgttggtgggcgggaatcaagcaggaatttggaattccctacaatccccaaagtcaaggagtagtagaatctatgaataaagaattaaagaaaattataggacaggtaagagatcaggctgaacatcttaagacagcagtacaaatggcagtattcatccacaattttaaaagaaaaggggggattggggggtacagtgcaggggaaagaatagtagacataatagcaacagacatacaaactaaagaattacaaaaacaaattacaaaaattcaaaattttcgggtttattacagggacagcagaaatccactttggaaaggaccagcaaagctcctctggaaaggtgaaggggcagtagtaatacaagataatagtgacataaaagtagtgccaagaagaaaagcaaagatcattagggattatggaaaacagatggcaggtgatgattgtgtggcaagtagacaggatgaggattagaacatggaaaagtttagtaaaacaccatatgtatgtttcagggaaagctaggggatggttttatagacatcactatgaaagccctcatccaagaataagttcagaagtacacatcccactaggggatgctagattggtaataacaacatattggggtctgcatacaggagaaagagactggcatttgggtcagggagtctccatagaatggaggaaaaagagatatagcacacaagtagaccctgaactagcagaccaactaattcatctgtattactttgactgtttttcagactctgctataagaaaggccttattaggacacatagttagccctaggtgtgaatatcaagcaggacataacaaggtaggatctctacaatacttggcactagcagcattaataacaccaaaaaagataaagccacctttgcctagtgttacgaaactgacagaggatagatggaacaagccccagaagaccaagggccacagagggagccacacaatgaatggacactagagcttttagaggagcttaagaatgaagctgttagacattttcctaggatttggctccatggcttagggcaacatatctatgaaacttatggggatacttgggcaggagtggaagccataataagaattctgcaacaactgctgtttatccattttcagaattgggtgtcgacatagcagaataggcgttactcgacagaggagagcaagaaatggagccagtagatcctagactagagccctggaagcatccaggaagtcagcctaaaactgcttgtaccaattgctattgtaaaaagtgttgctttcattgccaagtttgtttcataacaaaagccttaggcatctcctatggcaggaagaagcggagacagcgacgaagagctcatcagaacagtcagactcatcaagcttctctatcaaagcagtaagtagtacatgtaacgcaacctataccaatagtagcaatagtagcattagtagtagcaataataatagcaatagttgtgtggtccatagtaatcatagaatataggaaaatattaagacaaagaaaaatagacaggttaattgatagactaatagaaagagcagaagacagtggcaatgagagtgaaggagaaatatcagcacttgtggagatgggggtggagatggggcaccatgctccttgggatgttgatgatctgtagtgctacagaaaaattgtgggtcacagtctattatggggtacctgtgtggaaggaagcaaccaccactctattttgtgcatcagatgctaaagcatatgatacagaggtacataatgtttgggccacacatgcctgtgtacccacagaccccaacccacaagaagtagtattggtaaatgtgacagaaaattttaacatgtggaaaaatgacatggtagaacagatgcatgaggatataatcagtttatgggatcaaagcctaaagccatgtgtaaaattaaccccactctgtgttagtttaaagtgcactgatttgaagaatgatactaataccaatagtagtagcgggagaatgataatggagaaaggagagataaaaaactgctctttcaatatcagcacaagcataagaggtaaggtgcagaaagaatatgcatttttttataaacttgatataataccaatagataatgatactaccagctataagttgacaagttgtaacacctcagtcattacacaggcctgtccaaaggtatcctttgagccaattcccatacattattgtgccccggctggttttgcgattctaaaatgtaataataagacgttcaatggaacaggaccatgtacaaatgtcagcacagtacaatgtacacatggaattaggccagtagtatcaactcaactgctgttaaatggcagtctagcagaagaagaggtagtaattagatctgtcaatttcacggacaatgctaaaaccataatagtacagctgaacacatctgtagaaattaattgtacaagacccaacaacaatacaagaaaaagaatccgtatccagagaggaccagggagagcatttgttacaataggaaaaataggaaatatgagacaagcacattgtaacattagtagagcaaaatggaataacactttaaaacagatagctagcaaattaagagaacaatttggaaataataaaacaataatctttaagcaatcctcaggaggggacccagaaattgtaacgcacagttttaattgtggaggggaatttttctactgtaattcaacacaactgtttaatagtacttggtttaatagtacttggagtactgaagggtcaaataacactgaaggaagtgacacaatcaccctcccatgcagaataaaacaaattataaacatgtggcagaaagtaggaaaagcaatgtatgcccctcccatcagtggacaaattagatgttcatcaaatattacagggctgctattaacaagagatggtggtaatagcaacaatgagtccgagatcttcagacctggaggaggagatatgagggacaattggagaagtgaattatataaatataaagtagtaaaaattgaaccattaggagtagcacccaccaaggcaaagagaagagtggtgcagagagaaaaaagagcagtgggaataggagctttgttccttgggttcttgggagcagcaggaagcactatgggcgcagcctcaatgacgctgacggtacaggccagacaattattgtctggtatagtgcagcagcagaacaatttgctgagggctattgaggcgcaacagcatctgttgcaactcacagtctggggcatcaagcagctccaggcaagaatcctggctgtggaaagatacctaaaggatcaacagctcctggggatttggggttgctctggaaaactcatttgcaccactgctgtgccttggaatgctagttggagtaataaatctctggaacagatttggaatcacacgacctggatggagtgggacagagaaattaacaattacacaagcttaatacactccttaattgaagaatcgcaaaaccagcaagaaaagaatgaacaagaattattggaattagataaatgggcaagtttgtggaattggtttaacataacaaattggctgtggtatataaaattattcataatgatagtaggaggcttggtaggtttaagaatagtttttgctgtactttctatagtgaatagagttaggcagggatattcaccattatcgtttcagacccacctcccaaccccgaggggacccgacaggcccgaaggaatagaagaagaaggtggagagagagacagagacagatccattcgattagtgaacggatccttggcacttatctgggacgatctgcggagcctgtgcctcttcagctaccaccgcttgagagacttactcttgattgtaacgaggattgtggaacttctgggacgcagggggtgggaagccctcaaatattggtggaatctcctacagtattggagtcaggaactaaagaatagtgctgttagcttgctcaatgccacagccatagcagtagctgaggggacagatagggttatagaagtagtacaaggagcttgtagagctattcgccacatacctagaagaataagacagggcttggaaaggattttgctataagatgggtggcaagtggtcaaaaagtagtgtgattggatggcctactgtaagggaaagaatgagacgagctgagccagcagcagatagggtgggagcagcatctcgagacctggaaaaacatggagcaatcacaagtagcaatacagcagctaccaatgctgcttgtgcctggctagaagcacaagaggaggaggaggtgggttttccagtcacacctcaggtacctttaagaccaatgacttacaaggcagctgtagatcttagccactttttaaaagaaaaggggggactggaagggctaattcactcccaaagaagacaagatatccttgatctgtggatctaccacacacaaggctacttccctgattagcagaactacacaccagggccaggggtcagatatccactgacctttggatggtgctacaagctagtaccagttgagccagataagatagaagaggccaataaaggagagaacaccagcttgttacaccctgtgagcctgcatgggatggatgacccggagagagaagtgttagagtggaggtttgacagccgcctagcatttcatcacgtggcccgagagctgcatccggagtacttcaagaactgctgacatcgagcttgctacaagggactttccgctggggactttccagggaggcgtggcctgggcgggactggggagtggcgagccctcagatcctgcatataagcagctgctttttgcctgtactgggtctctctggttagaccagatctgagcctgggagctctctggctaactagggaacccactgcttaagcctcaataaagcttgccttgagtgcttcaagtagtgtgtgcccgtctgttgtgtgactctggtaactagagatccctcagacccttttagtcagtgtggaaaatctctagca

SEQ ID NO: 5 - DNA, 3506 bp, Human immunodeficiency virus
  MISC_FEATURE (1)..(650): HXB2 Protease gene nt 1900 through 2549
  MISC_FEATURE (651)..(2336): HXB2 RT gene nt 2550 through 4229
  MISC_FEATURE (2337)..(3506): HXB2 INT gene nt 4230 through 5400
acaaattcagctaccataatgatgcagagaggcaattttaggaaccaaagaaagattgttaagtgtttcaattgtggcaaagaagggcacacagccagaaattgcagggcccctaggaaaaagggctgttggaaatgtggaaaggaaggacaccaaatgaaagattgtactgagagacaggctaattttttagggaagatctggccttcctacaagggaaggccagggaattttcttcagagcagaccagagccaacagccccaccagaagagagcttcaggtctggggtagagacaacaactccccctcagaagcaggagccgatagacaaggaactgtatcctttaacttccctcaggtcactctttggcaacgacccctcgtcacaataaagataggggggcaactaaaggaagctctaatataaacaggagcagataatacaatattagaagaaatgagtttgccaggaagatggaaaccaaaaatactagtgggagttggaggttttatgaaagtaagacagtatgatcagatactcatagaaatctgtggacataaagctatatctacagtagtagtaggacctacacctgccaacgtaattggaagagatctgatgactcagattggttgcactttaaattttcccattagccctattgagactgtaccagtaaaattaaagccaggaatggatggcccaaaagttaaacaatggccattgacagaagaaaaaataaaagcattagtagaaatttgtacagagttggaaaaggaagggaaaatttcaaaaattgggcctgaaaatccatacaatactccagtatttgccataaagagaaaaaacagttcttcctccagatggagaaaagtagtagatctcagagaacttaataagagaactcaagacttctgggaagttcaattaggaataccacatcccgcagggatagaaaagaacaaatcagcaacaatactgtaagtgggtgatgcattttattcagttcccttagatgaagacttcaggaagtatactgcatttaccatacctagtataaacaatgagacaccagggattagatatcagtacaatgtgcttccaatgggatggaaaggatcaccagcaatattccaaagtagcatgacaaaaatcttagagccttttagaaaacaaaatccagacatagttatctgtcaatacgtggatgatttgttagtagcatctgacttagaaatagggcagcatagaacaaaaatagaggagctgagacaacatctgtggaggtggggactttacacaccagaccaaaaacatcagaaagaacatccattcctttggctgggttatgaactccatcctgataaatggacagtacagcctatagtgctgccagaaaaagacagctggactgtcaatgacatacagaagttagtggggaaattgaattgggcaagtcagatttacccagggattaaagtaaggcaattatgtaaactccttagaggaaccaaagcactaacagaagtaataccactaacagaagaagcagagctagaactggcagaaaacagagagattctaaaagaaccagtacatggagtgtattatgacccatcaaaagacttaatagcagaaatacagaagcaggggcaaggccaatggacatatcaaatttatcaagagccatttaaaaatctgaaaacaggaaaatatgcaagaatgaggggtgcccacactaatgatgtaaaacaattaacagaggcagtgcaaaaaataaccacagaaagcatagtaatatggggaaagactcctaaatttaaactgcccatacaaaaggaaacatgggaaacatggtggacagagtattggcaagccacctggattcctgagtgggagtttgttaatacccctcccttagtgaaattatggtaccagttagagaaagaacccatagtaggagcagaaaccttctatgtagatggggcagctaacagggagactaaattaggaaaagcaggatatgttactaatagaggaagacaaaaagttgtcaccctaactgacacaacaaatcagaagactgagttacaagcaatttatctagctttgcaggattcgggattagaagtaaacatagtaacagactcacaatatgcattaggaatcattcaagcacaaccagatcaaagtgaatcagagttagtcaatcaaataatagagcagttaataaaaaaggaaaaggtctatctggcatgggtaccagcacacaaaggaattggaggaaatgaacaagtagataaattagtcagtgctggaatcaggaaagtactatttttagatggaatagataaggcccaagatgaacatgagaaatatcacagtaattggagagcaatggctagtgattttaacctgccacctgtagtagcaaaagaaatagtagccagctgtgataaatgtcagctaaaaggagaagccatgcatggacaagtagactgtagtccaggaatatggcaactagattgtatacatttagaaggaaaagttatcatggtagcagttcatgtagccagtggatatatagaagcagaagttattccagcacaaacagggcaggaagcagcatattttcttttaaaattagcaggaagatggccagtaaaaacaatacatactgacaatggcagcaatttcaccggtgctacggttagggccgcctgttggtgggcgggaatcaagcaggcattttcaattccccgcaatccccaaagtcacggagtagtataatctatgcataaagaattaaagaaaattataggacaggtaagagatcaggctgaacatcttaagacagcagtacaaatggcagtattcatccacaattttaaaagaaaaggggggattggggggtacagtgcaggggaaagaatagtagacataatagcaacagacatacaaactaaagaattacaaaaacaaattacaaaaattcaaaattttcgggtttattacagggacagcagaaatccactttggaaaggaccagcaaagctcctctggaaaggtgaaggggcagtagtaatacaagataatagtgacataaaagtagtgccaagaagaaaagcaaagatcattagggattatggaaaacagatggcaggtgatgattgtgtggcaagtagacaggatgaggattagaacatggaaaagtttagtaaaacaccatatgtatgtttcagggaaagctaggggatggttttatagacatcactatgaaagccctcatccaagaataagttcagaagtacacatcccactaggggatgctagattggtaataacaacatattggggtctgcatacaggagaaagagactggcatttgggtcagggagtctccatagaatggaggaaaaagagatatagcacacaagtagaccctgaactagcagaccaactaattcatctgtattactttgactgtttttcagactctgctat

SEQ ID NO: 6 - DNA, 3500 bp, Human immunodeficiency virus
  MISC_FEATURE (1)..(650): HXB2 Protease gene nt 1900 through 2549
  MISC_FEATURE (651)..(2330): HXB2 RT gene nt 2550 through 4229
  MISC_FEATURE (2331)..(3500): HXB2 INT gene nt 4230 through 5400
acaaattcagctaccataatgatgcagagaggcaattttaggaaccaaagaaagattgttaagtgtttcaattgtggcaaagaagggcacacagccagaaattgcagggcccctaggaaaaagggctgttggaaatgtggaaaggaaggacaccaaatgaaagattgtactgagagacaggctaattttttagggaagatctggccttcctacaagggaaggccagggaattttcttcagagcagaccagagccaacagccccaccagaagagagcttcaggtctggggtagagacaacaactccccctcagaagcaggagccgatagacaaggaactgtatcctttaacttccctcaggtcactctttggcaacgacccctcgtcacaataaagataggggggcaactaaaggaagctctattataaacaggagcagatgatacagtattagaagaaatgagtttgccaggaagatggaaaccaaaaatgatagggggaattggaggttttatcaaagtaagacagtatgatcagatactcatagaaatctgtggacataaagctataggtacagtattagtaggacctacacctgtcaacataattggaagaaatctgttgactcagattggttgcactttaaattttcccattagccctattgagactgtaccagtaaaattaaagccaggaatggatggcccaaaagttaaacaatggccattgacagaagaaaaaataaaagcattagtagaaatttgtacagagatggaaaaggaagggaaaatttcaaaaattgggcctgaaaatccatacaatactccagtatttgccataaagaaaaaagacagtactaaatggagaaaattagtagatttcagagaacttaataagagaactcaagacttctgggaagttcaattaggaataccacatcccgcagggttaaaaaagaaaaaatcagtaacagtactgtaagtgggtgatgcatatttttcagttcccttagatgaagacttcaggaagtatactgcatttaccatacctagtataaacaatgagacaccagggattagatatcagtacaatgtgcttccacagggatggaaaggatcaccagcaatattccaaagtagcatgacaaaaatcttagagccttttagaaaacaaaatccagacatagttatctatcaatacatggatgatttgtatgtaggatctgacttagaaatagggcagcatagaacaaaaatagaggagctgagacaacatctgttgaggtggggacttaccacaccagacaaaaaacatcagaaagaacctccattcctttggatgggttatgaactccatcctgataaatggacagtacagcctatagtgctgccagaaaaagacagctggactgtcaatgacatacagaagttagtggggaaattgaattgggcaagtcagatttacccagggattaaagtaaggcaattatgtaaactccttagaggaaccaaagcactaacagaagtaataccactaacagaagaagcagagctagaactggcagaaaacagagagattctaaaagaaccagtacatggagtgtattatgacccatcaaaagacttaatagcagaaatacagaagcaggggcaaggccaatggacatatcaaatttatcaagagccatttaaaaatctgaaaacaggaaaatatgcaagaatgaggggtgcccacactaatgatgtaaaacaattaacagaggcagtgcaaaaaataaccacagaaagcatagtaatatggggaaagactcctaaatttaaactgcccatacaaaaggaaacatgggaaacatggtggacagagtattggcaagccacctggattcctgagtgggagtttgttaatacccctcccttagtgaaattatggtaccagttagagaaagaacccatagtaggagcagaaaccttctatgtagatggggcagctaacagggagactaaattaggaaaagcaggatatgttactaatagaggaagacaaaaagttgtcaccctaactgacacaacaaatcagaagactgagttacaagcaatttatctagctttgcaggattcgggattagaagtaaacatagtaacagactcacaatatgcattaggaatcattcaagcacaaccagatcaaagtgaatcagagttagtcaatcaaataatagagcagttaataaaaaaggaaaaggtctatctggcatgggtaccagcacacaaaggaattggaggaaatgaacaagtagataaattagtcagtgctggaatcaggaaagtactatttttagatggaatagataaggcccaagatgaacatgagaaatatcacagtaattggagagcaatggctagtgattttaacctgccacctgtagtagcaaaagaaatagtagccagctgtgataaatgtcagctaaaaggagaagccatgcatggacaagtagactgtagtccaggaatatggcaactagattgtacacatttagaaggaaaagttatcctggtagcagttcatgtagccagtggatatatagaagcagaagttattccagcagaaacagggcaggaaacagcatattttcttttaaaattagcaggaagatggccagtaaaaacaatacatactgacaatggcagcaatttcaccggtgctacggttagggccgcctgttggtgggcgggaatcaagcaggaatttggaattccctacaatccccaaagtcaaggagtagtataatctatgaataaagaattaaagaaaattataggacaggtaagagatcaggctgaacatcttaagacagcagtacaaatggcagtattcatccacaattttaaaagaaaaggggggattggggggtacagtgcaggggaaagaatagtagacataatagcaacagacatacaaactaaagaattacaaaaacaaattacaaaaattcaaaattttcgggtttattacagggacagcagaaatccactttggaaaggaccagcaaagctcctctggaaaggtgaaggggcagtagtaatacaagataatagtgacataaaagtagtgccaagaagaaaagcaaagatcattagggattatggaaaacagatggcaggtgatgattgtgtggcaagtagacaggatgaggattagaacatggaaaagtttagtaaaacaccatatgtatgtttcagggaaagctaggggatggttttatagacatcactatgaaagccctcatccaagaataagttcagaagtacacatcccactaggggatgctagattggtaataacaacatattggggtctgcatacaggagaaagagactggcatttgggtcagggagtctccatagaatggaggaaaaagagatatagcacacaagtagaccctgaactagcagaccaactaattcatctgtattactttgactgtttttcagactctgctat

SEQ ID NO: 7 - DNA, 1526 bp, Human immunodeficiency virus
atgatctgtagtgctacagaaaaattgtgggtcacagtctattatggggtacctgtgtggaaggaagcaaccaccactctattttgtgcatcagatgctaaagcatatgatacagaggtacataatgtttgggccacacatgcctgtgtacccacagaccccaacccacaagaagtagtattggtaaatgtgacagaaaattttaacatgtggaaaaatgacatggtagaacagatgcatgaggatataatcagtttatgggatcaaagcctaaagccatgtgtaaaattaaccccactctgtgttagtttaaagtgcactgatttgaagaatgatactaataccaatagtagtagcgggagaatgataatggagaaaggagagataaaaaactgctctttcaatatcagcacaagcataagaggtaaggtgcagaaagaatatgcatttttttataaacttgatataataccaatagataatgatactaccagctataagttgacaagttgtaacacctcagtcattacacaggcctgtccaaaggtatcctttgagccaattcccatacattattgtgccccggctggttttgcgattctaaaatgtaataataagacgttcaatggaacaggaccatgtacaaatgtcagcacagtacaatgtacacatggaattaggccagtagtatcaactcaactgctgttaaatggcagtctagcagaagaagaggtagtaattagatctgtcaatttcacggacaatgctaaaaccataatagtacagctgaacacatctgtagaaattaattgtacaagacccaacaacaatacaagaaaaagaatccgtatccagagaggaccagggagagcatttgttacaataggaaaaataggaaatatgagacaagcacattgtaacattagtagagcaaaatggaataacactttaaaacagatagctagcaaattaagagaacaatttggaaataataaaacaataatctttaagcaatcctcaggaggggacccagaaattgtaacgcacagttttaattgtggaggggaatttttctactgtaattcaacacaactgtttaatagtacttggtttaatagtacttggagtactgaagggtcaaataacactgaaggaagtgacacaatcaccctcccatgcagaataaaacaaattataaacatgtggcagaaagtaggaaaagcaatgtatgcccctcccatcagtggacaaattagatgttcatcaaatattacagggctgctattaacaagagatggtggtaatagcaacaatgagtccgagatcttcagacctggaggaggagatatgagggacaattggagaagtgaattatataaatataaagtagtaaaaattgaaccattaggagtagcacccaccaaggcaaagagaagagtggtgcagagagaaaaaagagcagtgggaataggagctttgttccttgggttcttgggagcagcaggaagcactatgggcgcagcctc

SEQ ID NO: 8 - DNA, 1520 bp, Human immunodeficiency virus
atgatctgtagtgctacagaaaaattgtgggtcacagtctattatggggtacctgtgtggaaagaagcaaccaccactctattttgtgcatcagatgctaaagcatatgatacagaggtacataatgtttgggccacacatgcctgtgtacccacagaccccaacccacaagaagtagaattggaaaatgtgacagaaaattttaacatgtggaaaaataacatggtagaacagatgcatgaggatataatcagtttatgggatcaaagcctaaagccatgtgtaaaattaactccactctgtgttactttaaattgcactgatttgaggaatgctactaatgggaatgacactaataccactagtagtagcagggaaatgatggggggaggagaaatgaaaaattgctctttcaaaatcaccacaaacataagaggtaaggtgcagaaagaatatgcacttttttataaacttgatatagtaccaatagataataatagtaataatagatataggttgataagttgtaacacctcagtcattacacaggcctgtccaaagatatcctttgagccaattcccatacattattgtgccccggctggttttgcgattctaaagtgtaaagataagaagttcaatggaaaaggaccatgttcaaatgtcagcacagtacaatgtacacatgggattaggccagtagtatcaactcaactgctgttaaatggcagtctagcagaagaagaggtagtaattagatccgaaaatttcgcggacaatgctaaaaccataatagtacagctgaatgaatctgtagaaattaattgtacaagacccaacaacaatacaagaaaaagtatacatataggaccaggcagagcattatatacaacaggaaaaataataggagatataagacaagcacattgtaaccttagtagagcaaaatggaatgacactttaaataaaatagttataaaattaagagaacaatttgggaataaaacaatagtctttaagcattcctcaggaggggacccagaaattgtgacgcacagttttaattgtggaggggaatttttctactgtaattcaacacaactgtttaatagtacttggaatgttactgaagagtcaaataacactgtagaaaataacacaatcacactcccatgcagaataaaacaaattataaacatgtggcagaaagtaggaagagcaatgtatgcccctcccatcagaggacaaattagatgttcatcaaatattacagggctgctattaacaagagatggtggtccagaggacaacaagaccgaggtcttcagacctggaggaggagatatgagggacaattggagaagtgaattatataaatataaagtagtaaaaattgaaccattaggagtagcacccaccaaggcaaagagaagagtggtgcagagagaaaaaagagcagtgggaataggagctgtgttccttgggttcttgggagcagcaggaagcactatgggcgcagc

SEQ ID NO: 9 - DNA, 10080 bp, Artificial Sequence
  Description of Artificial Sequence: Synthetic polynucleotide
  MISC_FEATURE (1)..(7652): Sindbis gene sequence
  MISC_FEATURE (7653)..(9707): Ebola GP insert sequence
  MISC_FEATURE (9708)..(10080): Sindbis gene sequence
attgacggcgtagtacacactattgaatcaaacagccgaccaattgcactaccatcacaatggagaagccagtagtaaacgtagacgtagacccccagagtccgtttgtcgtgcaactgcaaaaaagcttcccgcaatttgaggtagtagcacagcaggtcactccaaatgaccatgctaatgccagagcattttcgcatctggccagtaaactaatcgagctggaggttcctaccacagcgacgatcttggacataggcagcgcaccggctcgtagaatgttttccgagcaccagtatcattgtgtctgccccatgcgtagtccagaagacccggaccgcatgatgaaatacgccagtaaactggcggaaaaagcgtgcaagattacaaacaagaacttgcatgagaagattaaggatctccggaccgtacttgatacgccggatgctgaaacaccatcgctctgctttcacaacgatgttacctgcaacatgcgtgccgaatattccgtcatgcaggacgtgtatatcaacgctcccggaactatctatcatcaggctatgaaaggcgtgcggaccctgtactggattggcttcgacaccacccagttcatgttctcggctatggcaggttcgtaccctgcgtacaacaccaactgggccgacgagaaagtccttgaagcgcgtaacatcggactttgcagcacaaagctgagtgaaggtaggacaggaaaattgtcgataatgaggaagaaggagttgaagcccgggtcgcgggtttatttctccgtaggatcgacactttatccagaacacagagccagcttgcagagctggcatcttccatcggtgttccacttgaatggaaagcagtcgtacacttgccgctgtgatacagtggtgagttgcgaaggctacgtagtgaagaaaatcaccatcagtcccgggatcacgggagaaaccgtgggatacgcggttacacacaatagcgagggcttcttgctatgcaaagttactgacacagtaaaaggagaacgggtatcgttccctgtgtgcacgtacatcccggccaccatatgcgatcagatgactggtataatggccacggatatatcacctgacgatgcacaaaaacttctggttgggctcaaccagcgaattgtcattaacggtaggactaacaggaacaccaacaccatgcaaaattaccttctgccgatcatagcacaagggttcagcaaatgggctaaggagcgcaaggatgatcttgataacgagaaaatgctgggtactagagaacgcaagcttacgtatggctgcttgtgggcgtttcgcactaagaaagtacattcgttttatcgcccacctggaacgcagacctgcgtaaaagtcccagcctcttttagcgcttttcccatgtcgtccgtatggacgacctctttgcccatgtcgctgaggcagaaattgaaactggcattgcaaccaaagaaggaggaaaaactgctgcaggtctcggaggaattagtcatggaggccaaggctgcttttgaggatgctcaggaggaagccagagcggagaagctccgagaagcacttccaccattagtggcagacaaaggcatcgaggcagccgcagaagttgtctgcgaagtggaggggctccaggcggacatcggagcagcattagttgaaaccccgcgcggtcacgtaaggataatacctcaagcaaatgaccgtatgatcggacagtatatcgttgtctcgccaaactctgtgctgaagaatgccaaactcgcaccagcgcacccgctagcagatcaggttaagatcataacacactccggaagatcaggaaggtacgcggtcgaaccatacgacgctaaagtactgatgccagcaggaggtgccgtaccatggccagaattcctagcactgagtgagagcgccacgttagtgtacaacgaaagagagtttgtgaaccgcaaactataccacattgccatgcatggccccgccaagaatacagaagaggagcagtacaaggttacaaaggcagagcttgcagaaacagagtacgtgtttgacgtggacaagaagcgttgcgttaagaaggaagaagcctcaggtctggtcctctcgggagaactgaccaaccctccctatcatgagctagctctggagggactgaagacccgacctgcggtcccgtacaaggtcgaaacaataggagtgataggcacaccggggtcgggcaagtcagctattatcaagtcaactgtcacggcacgagatcttgttaccagcggaaagaaagaaaattgtcgcgaaattgaggccgacgtgctaagactgaggggtatgcagattacgtcgaagacagtagattcggttatgctcaacggatgccacaaagccgtagaagtgctgtacgttgacgaagcgttcgcgtgccacgcaggagcactacttgccttgattgctatcgtcaggccccgcaagaaggtagtactatgcggagaccccatgcaatgcggattcttcaacatgatgcaactaaaggtacatttcaatcaccctgaaaaagacatatgcaccaagacattctacaagtatatctcccggcgttgcacacagccagttacagctattgtatcgacactgcattacgatggaaagatgaaaaccacgaacccgtgcaagaagaacattgaaatcgatattacaggggccacaaagccgaagccaggggatatcatcctgacatgtttccgcgggtgggttaagcaattgcaaatcgactatcccggacatgaagtaatgacagccgcggcctcacaagggctaaccagaaaaggagtgtatgccgtccggcaaaaagtcaatgaaaacccactgtacgcgatcacatcagagcatgtgaacgtgttgctcacccgcactgaggacaggctagtgtggaaaaccttgcagggcgacccatggattaagcagcccactaacatacctaaaggaaactttcaggctactatagaggactgggaagctgaacacaagggaataattgctgcaataaacagccccactccccgtgccaatccgttcagctgcaagaccaacgtttgctgggcgaaagcattggaaccgatactagccacggccggtatcgtacttaccggttgccagtggagcgaactgttcccacagtttgcggatgacaaaccacattcggccatttacgccttagacgtaatttgcattaagtttttcggcatggacttgacaagcggactgttttctaaacagagcatcccactaacgtaccatcccgccgattcagcgaggccggtagctcattgggacaacagcccaggaacccgcaagtatgggtacgatcacgccattgccgccgaactctcccgtagatttccggtgttccagctagctgggaagggcacacaacttgatttgcagacggggagaaccagagttatctctgcacagcataacctggtcccggtgaaccgcaatcttcctcacgccttagtccccgagtacaaggagaagcaacccggcccggtcaaaaaattcttgaaccagttcaaacaccactcagtacttgtggtatcagaggaaaaaattgaagctccccgtaagagaatcgaatggatcgccccgattggcatagccggtgcagataagaactacaacctggctttcgggtttccgccgcaggcacggtacgacctggtgttcatcaacattggaactaaatacagaaaccaccactttcagcagtgcgaagaccatgcggcgaccttaaaaaccctttcgcgttcggccctgaattgccttaacccaggaggcaccctcgtggtgaagtcctatggctacgccgaccgcaacagtgaggacgtagtcaccgctcttgccagaaagtttgtcagggtgtctgcagcgagaccagattgtgtctcaagcaatacagaaatgtacctgattttccgacaactagacaacagccgtacacggcaattcaccccgcaccatctgaattgcgtgatttcgtccgtgtatgagggtacaagagatggagttggagccgcgccgtcataccgcaccaaaagggagaatattgctgactgtcaagaggaagcagttgtcaacgcagccaatccgctgggtagaccaggcgaaggagtctgccgtgccatctataaacgttggccgaccagttttaccgattcagccacggagacaggcaccgcaagaatgactgtgtgcctaggaaagaaagtgatccacgcggtcggccctgatttccggaagcacccagaagcagaagccttgaaattgctacaaaacgcctaccatgcagtggcagacttagtaaatgaacataacatcaagtctgtcgccattccactgctatctacaggcatttacgcagccggaaaagaccgccttgaagtatcacttaactgcttgacaaccgcgctagacagaactgacgcggacgtaaccatctattgcctggataagaagtggaaggaaagaatcgacgcggcactccaacttaaggagtctgtaacagagctgaaggatgaagatatggagatcgacgatgagttagtatggattcatccagacagttgcttgaagggaagaaagggattcagtactacaaaaggaaaattgtattcgtacttcgaaggcaccaaattccatcaagcagcaaaagacatggcggagataaaggtcctgttccctaatgaccaggaaagtaatgaacaactgtgtgcctacatattgggtgagaccatggaagcaatccgcgaaaagtgcccggtcgaccataacccgtcgtctagcccgcccaaaacgttgccgtgcctttgcatgtatgccatgacgccagaaagggtccacagacttagaagcaataacgtcaaagaagttacagtatgctcctccaccccccttcctaagcacaaaattaagaatgttcagaaggttcagtgcacgaaagtagtcctgtttaatccgcacactcccgcattcgttcccgcccgtaagtacatagaagtgccagaacagcctaccgctcctcctgcacaggccgaggaggcccccgaagttgtagcgacaccgtcaccatctacagctgataacacctcgcttgatgtcacagacatctcactggatatggatgacagtagcgaaggctcacttttttcgagctttagcggatcggacaactctattactagtatggacagttggtcgtcaggacctagttcactagagatagtagaccgaaggcaggtggtggtggctgacgttcatgccgtccaagagcctgcccctattccaccgccaaggctaaagaagatggcccgcctggcagcggcaagaaaagagcccactccaccggcaagcaatagctctgagtccctccacctctcttttggtggggtatccatgtccctcggatcaattttcgacggagagacggcccgccaggcagcggtacaacccctggcaacaggccccacggatgtgcctatgtctttcggatcgttttccgacggagagattgatgagctgagccgcagagtaactgagtccgaacccgtcctgtttggatcatttgaaccgggcgaagtgaactcaattatatcgtcccgatcagccgtatcttttccactacgcaagcagagacgtagacgcaggagcaggaggactgaatactgactaaccggggtaggtgggtacatattttcgacggacacaggccctgggcacttgcaaaagaagtccgttctgcagaaccagcttacagaaccgaccttggagcgcaatgtcctggaaagaattcatgccccggtgctcgacacgtcgaaagaggaacaactcaaactcaggtaccagatgatgcccaccgaagccaacaaaagtaggtaccagtctcgtaaagtagaaaatcagaaagccataaccactgagcgactactgtcaggactacgactgtataactctgccacagatcagccagaatgctataagatcacctatccgaaaccattgtactccagtagcgtaccggcgaactactccgatccacagttcgctgtagctgtctgtaacaactatctgcatgagaactatccgacagtagcatcttatcagattactgacgagtacgatgcttacttggatatggtagacgggacagtcgcctgcctggatactgcaaccttctgccccgctaagcttagaagttacccgaaaaaacatgagtatagagccccgaatatccgcagtgcggttccatcagcgatgcagaacacgctacaaaatgtgctcattgccgcaactaaaagaaattgcaacgtcacgcagatgcgtgaactgccaacactggactcagcgacattcaatgtcgaatgctttcgaaaatatgcatgtaatgacgagtattgggaggagttcgctcggaagccaattaggattaccactgagtttgtcaccgcatatgtagctagactgaaaggccctaaggccgccgcactatttgcaaagacgtataatttggtcccattgcaagaagtgcctatggatagattcgtcatggacatgaaaagagacgtgaaagttacaccaggcacgaaacacacagaagaaagaccgaaagtacaagtgatacaagccgcagaacccctggcgactgcttacttatgcgggattcaccgggaattagtgcgtaggcttacggccgtcttgcttccaaacattcacacgctttttgacatgtcggcggaggattttgatgcaatcatagcagaacacttcaagcaaggcgacccggtactggagacggatatcgcatcattcgacaaaagccaagacgacgctatggcgttaaccggtctgatgatcttggaggacctgggtgtggatcaaccactactcgacttgatcgagtgcgcctttggagaaatatcatccacccatctacctacgggtactcgttttaaattcggggcgatgatgaaatccggaatgttcctcacactttttgtcaacacagttttgaatgtcgttatcgccagcagagtactagaagagcggcttaaaacgtccagatgtgcagcgttcattggcgacgacaacatcatacatggagtagtatctgacaaagaaatggctgagaggtgcgccacctggctcaacatggaggttaagatcatcgacgcagtcatcggtgagagaccaccttacttctgcggcggatttatcttgcaagattcggttacttccacagcgtgccgcgtggcggatcccctgaaaaggctgtttaagttgggtaaaccgctcccagccgacgacgagcaagacgaagacagaagacgcgctctgctagatgaaacaaaggcgtggtttagagtaggtataacaggcactttagcagtggccgtgacgacccggtatgaggtagacaatattacacctgtcctactggcattgagaacttttgcccagagcaaaagagcattccaagccatcagaggggaaataaagcatctctacggtggtcctaaatagtcagcatagtacatttcatctgactaatactacaacaccaccacctctagatctagaaggaatattgcagttacctcgtgatcgattcaagaggacatcattctttctttgggtaattatccttttccaaagaacattttccatcccgcttggagttatccacaatagtacattacaggttagtgatgtcgacaaactagtttgtcgtgacaaactgtcatccacaaatcaattgagatcagttggactgaatctcgaggggaatggagtggcaactgacgtgccatctgcgactaaaagatggggcttcaggtccggtgtcccaccaaaggtggtcaattatgaagctggtgaatgggctgaaaactgctacaatcttgaaatcaaaaaacctgacgggagtgagtgtctaccagcagcgccagacgggattcggggcttcccccggtgccggtatgtgcacaaagtatcaggaacgggaccatgtgccggagactttgccttccacaaagagggtgctttcttcctgtatgatcgacttgcttccacagttatctaccgaggaacgactttcgctgaaggtgtcgttgcatttctgatactgccccaagctaagaaggacttcttcagctcacaccccttgagagagccggtcaatgcaacggaggacccgtcgagtggctattattctaccacaattagatatcaggctaccggttttggaactaatgagacagagtacttgttcgaggttgacaatttgacctacgtccaacttgaatcaagattcacaccacagtttctgctccagctgaatgagacaatatatgcaagtgggaagaggagcaacaccacgggaaaactaatttggaaggtcaaccccgaaattgatacaacaatcggggagtgggccttcagggaaactaaaaaaacctcactagaaaaattcgcagtgaagagttgtctttcacagctgtatcaaacggacccaaaaacatcagtggtcagagtccggcgcgaacttcttccgacccagagaccaacacaacaaatgaagaccacaaaatcatggcttcagaaaattcctctgcaatggttcaagtgcacagtcaaggaaggaaagctgcagtgtcgcatctgacaacccttgccacaatctccacgagtcctcaacctcccacaaccaaaacaggtccggacaacagcacccataatacacccgtgtataaacttgacatctctgaggcaactcaagttggacaacatcaccgtagagcagacaacgacagcacagcctccgacactccccccgccacgaccgcagccggacccttaaaagcagagaacaccaacacgagtaagagcgctgactccctggacctcgccaccacgataagcccccaaaactacagcgagactgctggcaacaacaacactcatcaccaagataccggagaagagagtgccagcagcgggaagctaggcttaattaccaatactattgctggagtagcaggactgatcacaggcgggagaaggactcgaagagaagtaattgtcaatgctcaacccaaatgcaaccccaatttacattactggactactcaggatgaaggtgctgcaatcggattggcctggataccatatttcgggccagcagccgaaggaatttacacagaggggctaatgcacaaccaagatggtttaatctgtgggttgaggcagctggccaacgaaacgactcaagctctccaactgttcctgagagccacaactgagctgcgaaccttttcaatcctcaaccgtaaggcaattgacttcctgctgcagcgatggggtggcacatgccacattttgggaccggactgctgtatcgaaccacatgattggaccaagaacataacagacaaaattgatcagattattcatgattttgttgataaaacccttccggaccagggggacaatgacaattggtggacaggatggagacaatggataccggcaatttaaatatcgagggcaggagcgagagggccaaggccagggagggcggccaccaccatcaccaccatcaccattagtaatgaggtaaccgtggggcccaatgatccgaccagcaaaactcgatgtacttccgaggaactgatgtgcataatgcatcaggctggtacattagatccccgcttaccgcgggcaatatagcaacactaaaaactcgatgtacttccgaggaagcgcagtgcataatgctgcgcagtgttgccacataaccactatattaaccatttatctagcggacgccaaaaactcaatgtatttctgaggaagcgtggtgcataatgccacgcagcgtctgcataacttttattatttcttttattaatcaacaaaattttgtttttaacatttcaaaaaaaaaaaaaaaaaaaaaaaaaaaaaaaaaaaaagggaattcctcgattaattaagcggccgc

SEQ ID NO: 10 - DNA, 10348 bp, Artificial Sequence
  Description of Artificial Sequence: Synthetic polynucleotide
  MISC_FEATURE (1)..(7652): Sindbis gene sequence
  MISC_FEATURE (7653)..(9975): Ebola NP/VP24 insert sequence
  MISC_FEATURE (9976)..(10348): Sindbis gene sequence
attgacggcgtagtacacactattgaatcaaacagccgaccaattgcactaccatcacaatggagaagccagtagtaaacgtagacgtagacccccagagtccgtttgtcgtgcaactgcaaaaaagcttcccgcaatttgaggtagtagcacagcaggtcactccaaatgaccatgctaatgccagagcattttcgcatctggccagtaaactaatcgagctggaggttcctaccacagcgacgatcttggacataggcagcgcaccggctcgtagaatgttttccgagcaccagtatcattgtgtctgccccatgcgtagtccagaagacccggaccgcatgatgaaatacgccagtaaactggcggaaaaagcgtgcaagattacaaacaagaacttgcatgagaagattaaggatctccggaccgtacttgatacgccggatgctgaaacaccatcgctctgctttcacaacgatgttacctgcaacatgcgtgccgaatattccgtcatgcaggacgtgtatatcaacgctcccggaactatctatcatcaggctatgaaaggcgtgcggaccctgtactggattggcttcgacaccacccagttcatgttctcggctatggcaggttcgtaccctgcgtacaacaccaactgggccgacgagaaagtccttgaagcgcgtaacatcggactttgcagcacaaagctgagtgaaggtaggacaggaaaattgtcgataatgaggaagaaggagttgaagcccgggtcgcgggtttatttctccgtaggatcgacactttatccagaacacagagccagcttgcagagctggcatcttccatcggtgttccacttgaatggaaagcagtcgtacacttgccgctgtgatacagtggtgagttgcgaaggctacgtagtgaagaaaatcaccatcagtcccgggatcacgggagaaaccgtgggatacgcggttacacacaatagcgagggcttcttgctatgcaaagttactgacacagtaaaaggagaacgggtatcgttccctgtgtgcacgtacatcccggccaccatatgcgatcagatgactggtataatggccacggatatatcacctgacgatgcacaaaaacttctggttgggctcaaccagcgaattgtcattaacggtaggactaacaggaacaccaacaccatgcaaaattaccttctgccgatcatagcacaagggttcagcaaatgggctaaggagcgcaaggatgatcttgataacgagaaaatgctgggtactagagaacgcaagcttacgtatggctgcttgtgggcgtttcgcactaagaaagtacattcgttttatcgcccacctggaacgcagacctgcgtaaaagtcccagcctcttttagcgcttttcccatgtcgtccgtatggacgacctctttgcccatgtcgctgaggcagaaattgaaactggcattgcaaccaaagaaggaggaaaaactgctgcaggtctcggaggaattagtcatggaggccaaggctgcttttgaggatgctcaggaggaagccagagcggagaagctccgagaagcacttccaccattagtggcagacaaaggcatcgaggcagccgcagaagttgtctgcgaagtggaggggctccaggcggacatcggagcagcattagttgaaaccccgcgcggtcacgtaaggataatacctcaagcaaatgaccgtatgatcggacagtatatcgttgtctcgccaaactctgtgctgaagaatgccaaactcgcaccagcgcacccgctagcagatcaggttaagatcataacacactccggaagatcaggaaggtacgcggtcgaaccatacgacgctaaagtactgatgccagcaggaggtgccgtaccatggccagaattcctagcactgagtgagagcgccacgttagtgtacaacgaaagagagtttgtgaaccgcaaactataccacattgccatgcatggccccgccaagaatacagaagaggagcagtacaaggttacaaaggcagagcttgcagaaacagagtacgtgtttgacgtggacaagaagcgttgcgttaagaaggaagaagcctcaggtctggtcctctcgggagaactgaccaaccctccctatcatgagctagctctggagggactgaagacccgacctgcggtcccgtacaaggtcgaaacaataggagtgataggcacaccggggtcgggcaagtcagctattatcaagtcaactgtcacggcacgagatcttgttaccagcggaaagaaagaaaattgtcgcgaaattgaggccgacgtgctaagactgaggggtatgcagattacgtcgaagacagtagattcggttatgctcaacggatgccacaaagccgtagaagtgctgtacgttgacgaagcgttcgcgtgccacgcaggagcactacttgccttgattgctatcgtcaggccccgcaagaaggtagtactatgcggagaccccatgcaatgcggattcttcaacatgatgcaactaaaggtacatttcaatcaccctgaaaaagacatatgcaccaagacattctacaagtatatctcccggcgttgcacacagccagttacagctattgtatcgacactgcattacgatggaaagatgaaaaccacgaacccgtgcaagaagaacattgaaatcgatattacaggggccacaaagccgaagccaggggatatcatcctgacatgtttccgcgggtgggttaagcaattgcaaatcgactatcccggacatgaagtaatgacagccgcggcctcacaagggctaaccagaaaaggagtgtatgccgtccggcaaaaagtcaatgaaaacccactgtacgcgatcacatcagagcatgtgaacgtgttgctcacccgcactgaggacaggctagtgtggaaaaccttgcagggcgacccatggattaagcagcccactaacatacctaaaggaaactttcaggctactatagaggactgggaagctgaacacaagggaataattgctgcaataaacagccccactccccgtgccaatccgttcagctgcaagaccaacgtttgctgggcgaaagcattggaaccgatactagccacggccggtatcgtacttaccggttgccagtggagcgaactgttcccacagtttgcggatgacaaaccacattcggccatttacgccttagacgtaatttgcattaagtttttcggcatggacttgacaagcggactgttttctaaacagagcatcccactaacgtaccatcccgccgattcagcgaggccggtagctcattgggacaacagcccaggaacccgcaagtatgggtacgatcacgccattgccgccgaactctcccgtagatttccggtgttccagctagctgggaagggcacacaacttgatttgcagacggggagaaccagagttatctctgcacagcataacctggtcccggtgaaccgcaatcttcctcacgccttagtccccgagtacaaggagaagcaacccggcccggtcaaaaaattcttgaaccagttcaaacaccactcagtacttgtggtatcagaggaaaaaattgaagctccccgtaagagaatcgaatggatcgccccgattggcatagccggtgcagataagaactacaacctggctttcgggtttccgccgcaggcacggtacgacctggtgttcatcaacattggaactaaatacagaaaccaccactttcagcagtgcgaagaccatgcggcgaccttaaaaaccctttcgcgttcggccctgaattgccttaacccaggaggcaccctcgtggtgaagtcctatggctacgccgaccgcaacagtgaggacgtagtcaccgctcttgccagaaagtttgtcagggtgtctgcagcgagaccagattgtgtctcaagcaatacagaaatgtacctgattttccgacaactagacaacagccgtacacggcaattcaccccgcaccatctgaattgcgtgatttcgtccgtgtatgagggtacaagagatggagttggagccgcgccgtcataccgcaccaaaagggagaatattgctgactgtcaagaggaagcagttgtcaacgcagccaatccgctgggtagaccaggcgaaggagtctgccgtgccatctataaacgttggccgaccagttttaccgattcagccacggagacaggcaccgcaagaatgactgtgtgcctaggaaagaaagtgatccacgcggtcggccctgatttccggaagcacccagaagcagaagccttgaaattgctacaaaacgcctaccatgcagtggcagacttagtaaatgaacataacatcaagtctgtcgccattccactgctatctacaggcatttacgcagccggaaaagaccgccttgaagtatcacttaactgcttgacaaccgcgctagacagaactgacgcggacgtaaccatctattgcctggataagaagtggaaggaaagaatcgacgcggcactccaacttaaggagtctgtaacagagctgaaggatgaagatatggagatcgacgatgagttagtatggattcatccagacagttgcttgaagggaagaaagggattcagtactacaaaaggaaaattgtattcgtacttcgaaggcaccaaattccatcaagcagcaaaagacatggcggagataaaggtcctgttccctaatgaccaggaaagtaatgaacaactgtgtgcctacatattgggtgagaccatggaagcaatccgcgaaaagtgcccggtcgaccataacccgtcgtctagcccgcccaaaacgttgccgtgcctttgcatgtatgccatgacgccagaaagggtccacagacttagaagcaataacgtcaaagaagttacagtatgctcctccaccccccttcctaagcacaaaattaagaatgttcagaaggttcagtgcacgaaagtagtcctgtttaatccgcacactcccgcattcgttcccgcccgtaagtacatagaagtgccagaacagcctaccgctcctcctgcacaggccgaggaggcccccgaagttgtagcgacaccgtcaccatctacagctgataacacctcgcttgatgtcacagacatctcactggatatggatgacagtagcgaaggctcacttttttcgagctttagcggatcggacaactctattactagtatggacagttggtcgtcaggacctagttcactagagatagtagaccgaaggcaggtggtggtggctgacgttcatgccgtccaagagcctgcccctattccaccgccaaggctaaagaagatggcccgcctggcagcggcaagaaaagagcccactccaccggcaagcaatagctctgagtccctccacctctcttttggtggggtatccatgtccctcggatcaattttcgacggagagacggcccgccaggcagcggtacaacccctggcaacaggccccacggatgtgcctatgtctttcggatcgttttccgacggagagattgatgagctgagccgcagagtaactgagtccgaacccgtcctgtttggatcatttgaaccgggcgaagtgaactcaattatatcgtcccgatcagccgtatcttttccactacgcaagcagagacgtagacgcaggagcaggaggactgaatactgactaaccggggtaggtgggtacatattttcgacggacacaggccctgggcacttgcaaaagaagtccgttctgcagaaccagcttacagaaccgaccttggagcgcaatgtcctggaaagaattcatgccccggtgctcgacacgtcgaaagaggaacaactcaaactcaggtaccagatgatgcccaccgaagccaacaaaagtaggtaccagtctcgtaaagtagaaaatcagaaagccataaccactgagcgactactgtcaggactacgactgtataactctgccacagatcagccagaatgctataagatcacctatccgaaaccattgtactccagtagcgtaccggcgaactactccgatccacagttcgctgtagctgtctgtaacaactatctgcatgagaactatccgacagtagcatcttatcagattactgacgagtacgatgcttacttggatatggtagacgggacagtcgcctgcctggatactgcaaccttctgccccgctaagcttagaagttacccgaaaaaacatgagtatagagccccgaatatccgcagtgcggttccatcagcgatgcagaacacgctacaaaatgtgctcattgccgcaactaaaagaaattgcaacgtcacgcagatgcgtgaactgccaacactggactcagcgacattcaatgtcgaatgctttcgaaaatatgcatgtaatgacgagtattgggaggagttcgctcggaagccaattaggattaccactgagtttgtcaccgcatatgtagctagactgaaaggccctaaggccgccgcactatttgcaaagacgtataatttggtcccattgcaagaagtgcctatggatagattcgtcatggacatgaaaagagacgtgaaagttacaccaggcacgaaacacacagaagaaagaccgaaagtacaagtgatacaagccgcagaacccctggcgactgcttacttatgcgggattcaccgggaattagtgcgtaggcttacggccgtcttgcttccaaacattcacacgctttttgacatgtcggcggaggattttgatgcaatcatagcagaacacttcaagcaaggcgacccggtactggagacggatatcgcatcattcgacaaaagccaagacgacgctatggcgttaaccggtctgatgatcttggaggacctgggtgtggatcaaccactactcgacttgatcgagtgcgcctttggagaaatatcatccacccatctacctacgggtactcgttttaaattcggggcgatgatgaaatccggaatgttcctcacactttttgtcaacacagttttgaatgtcgttatcgccagcagagtactagaagagcggcttaaaacgtccagatgtgcagcgttcattggcgacgacaacatcatacatggagtagtatctgacaaagaaatggctgagaggtgcgccacctggctcaacatggaggttaagatcatcgacgcagtcatcggtgagagaccaccttacttctgcggcggatttatcttgcaagattcggttacttccacagcgtgccgcgtggcggatcccctgaaaaggctgtttaagttgggtaaaccgctcccagccgacgacgagcaagacgaagacagaagacgcgctctgctagatgaaacaaaggcgtggtttagagtaggtataacaggcactttagcagtggccgtgacgacccggtatgaggtagacaatattacacctgtcctactggcattgagaacttttgcccagagcaaaagagcattccaagccatcagaggggaaataaagcatctctacggtggtcctaaatagtcagcatagtacatttcatctgactaatactacaacaccaccacctctagatctagaatactgtaatcatacctggtttgtttcagagccatatcaccaagatagagaacaacctaggtctccggagggggcaagggcatcagtgtgctcagttgaaaatcccttgtcaacatctaggccttatcacatcacaagttccgccttaaactctgcagggtgatccaacaaccttaatagcaacattattgttaaaggacagcattagttcacagtcaaacaagcaagattgagaattaactttgattttgaacctgaacacccagaggactggagactcaacaaccctaaagcctggggtaaaacattagaaatagtttaaagacaaattgctcggaatcacaaaattccgagtatggattctcgtcctcagaaagtctggtagacgccgagtctcactgaatctgacatggattaccacaagatcttgacagcaggtctgtccgttcaacaggggattgttcggcaaagagtcatcccagtgtatcaagtaaacaatcttgaggaaatttgccaacttatcatacaggcctttgaagctggtgttgattttcaagagagtgcggacagtttccttctcatgctttgtcttcatcatgcgtaccaaggagattacaaacttttcttggaaagtggcgcagtcaagtatttggaagggcacgggttccgttttgaagtcaagaagcgtgatggagtgaagcgccttgaggaattgctgccagcagtatctagtgggagaaacattaagagaacacttgctgccatgccggaagaggagacgacttaatgccggacatgatgccaacgatgctgtgatttcaaattcagtggctcaagctcgtttttcaggtctattgattgtcaaaacagtacttgatcatatcctacaaaagacagaacgaggagttcgtctccatcctcttgcaaggaccgccaaggtaaaaaatgaggtgaactccttcaaggctgcactcagctccctggccaagcatggagagtatgctcctttcgcccgacttttgaacctttctggagtaaataatcttgagcatggtcttttccctcaactgtcggcaattgcactcggagtcgccacagcccacgggagcaccctcgcaggagtaaatgttggagaacagtatcaacagctcagagaggcagccactgaggctgagaagcaactccaacaatatgcggagtctcgtgaacttgaccatcttggacttgatgatcaggaaaagaaaattcttatgaacttccatcagaaaaagaacgaaatcagcttccagcaaacaaacgcgatggtaactctaagaaaagagcgcctggccaagctgacagaagctatcactgctgcatcactgcccaaaacaagtggacattacgatgatgatgacgacattccctttccaggacccatcaatgatgacgacaatcctggccatcaagatgatgatccgactgactcacaggatacgaccattcccgatgtggtagttgatcccgatgatggaggctacggcgaataccaaagttactcggaaaacggcatgagtgcaccagatgacttggtcctatgtcttttagctgtataccagttgcccctgagatacgccacaaaagtgtctctgagctaaagtggtctgtacacatctcatacattgtattaggggcaataatatctaattgaacttagccatttaaaatttagtgcataaatctgggctaactccaccaggtcaactccattggctgaaaagaagcccacctacaacgaacattactttgagcgccctcacaattaaaaaataagagcgtcgttccaacaatcgagcgcaaggttacaaggttgaactgagagtgtctagacaacaaaatatcgatactccagacaccaagcaagacctgagaaaaaaccatggccaaagctacgggacgatacaatctaatatcgcccaaaaaggacctggagaaaggggttgtcttaagcgacctctgtaacttcttagttagtcaaactattcaagggtggaaagtttattgggctggtattgagtttgatgtgactcacaaaggaatggccctattgcatagactgaaaactaatgactttgcccctgcatggtcatggcggtgtttgcagatttggacctgcgagcgggttctgacctgaaggctctgcgcggacttgtggagacagccgctcaccttggctattatttaaatatcgagggcaggagcgagagggccaaggccagggagggcggccaccaccatcaccaccatcaccattagtaatgaggtaaccgtggggcccaatgatccgaccagcaaaactcgatgtacttccgaggaactgatgtgcataatgcatcaggctggtacattagatccccgcttaccgcgggcaatatagcaacactaaaaactcgatgtacttccgaggaagcgcagtgcataatgctgcgcagtgttgccacataaccactatattaaccatttatctagcggacgccaaaaactcaatgtatttctgaggaagcgtggtgcataatgccacgcagcgtctgcataacttttattatttcttttattaatcaacaaaattttgtttttaacatttcaaaaaaaaaaaaaaaaaaaaaaaaaaaaaaaaaaaaagggaattcctcgattaattaagcggccgc

SEQ ID NO: 11 - DNA, 11655 bp, Artificial Sequence
  Description of Artificial Sequence: Synthetic polynucleotide
  MISC_FEATURE (1)..(7646): Sindbis gene sequence
  MISC_FEATURE (7647)..(11166): Multi-mutant HIV-1 insert sequence
  MISC_FEATURE (11167)..(11655): Sindbis gene sequence
attgacggcgtagtacacactattgaatcaaacagccgaccaattgcactaccatcacaatggagaagccagtagtaaacgtagacgtagacccccagagtccgtttgtcgtgcaactgcaaaaaagcttcccgcaatttgaggtagtagcacagcaggtcactccaaatgaccatgctaatgccagagcattttcgcatctggccagtaaactaatcgagctggaggttcctaccacagcgacgatcttggacataggcagcgcaccggctcgtagaatgttttccgagcaccagtatcattgtgtctgccccatgcgtagtccagaagacccggaccgcatgatgaaatacgccagtaaactggcggaaaaagcgtgcaagattacaaacaagaacttgcatgagaagattaaggatctccggaccgtacttgatacgccggatgctgaaacaccatcgctctgctttcacaacgatgttacctgcaacatgcgtgccgaatattccgtcatgcaggacgtgtatatcaacgctcccggaactatctatcatcaggctatgaaaggcgtgcggaccctgtactggattggcttcgacaccacccagttcatgttctcggctatggcaggttcgtaccctgcgtacaacaccaactgggccgacgagaaagtccttgaagcgcgtaacatcggactttgcagcacaaagctgagtgaaggtaggacaggaaaattgtcgataatgaggaagaaggagttgaagcccgggtcgcgggtttatttctccgtaggatcgacactttatccagaacacagagccagcttgcagagctggcatcttccatcggtgttccacttgaatggaaagcagtcgtacacttgccgctgtgatacagtggtgagttgcgaaggctacgtagtgaagaaaatcaccatcagtcccgggatcacgggagaaaccgtgggatacgcggttacacacaatagcgagggcttcttgctatgcaaagttactgacacagtaaaaggagaacgggtatcgttccctgtgtgcacgtacatcccggccaccatatgcgatcagatgactggtataatggccacggatatatcacctgacgatgcacaaaaacttctggttgggctcaaccagcgaattgtcattaacggtaggactaacaggaacaccaacaccatgcaaaattaccttctgccgatcatagcacaagggttcagcaaatgggctaaggagcgcaaggatgatcttgataacgagaaaatgctgggtactagagaacgcaagcttacgtatggctgcttgtgggcgtttcgcactaagaaagtacattcgttttatcgcccacctggaacgcagacctgcgtaaaagtcccagcctcttttagcgcttttcccatgtcgtccgtatggacgacctctttgcccatgtcgctgaggcagaaattgaaactggcattgcaaccaaagaaggaggaaaaactgctgcaggtctcggaggaattagtcatggaggccaaggctgcttttgaggatgctcaggaggaagccagagcggagaagctccgagaagcacttccaccattagtggcagacaaaggcatcgaggcagccgcagaagttgtctgcgaagtggaggggctccaggcggacatcggagcagcattagttgaaaccccgcgcggtcacgtaaggataatacctcaagcaaatgaccgtatgatcggacagtatatcgttgtctcgccaaactctgtgctgaagaatgccaaactcgcaccagcgcacccgctagcagatcaggttaagatcataacacactccggaagatcaggaaggtacgcggtcgaaccatacgacgctaaagtactgatgccagcaggaggtgccgtaccatggccagaattcctagcactgagtgagagcgccacgttagtgtacaacgaaagagagtttgtgaaccgcaaactataccacattgccatgcatggccccgccaagaatacagaagaggagcagtacaaggttacaaaggcagagcttgcagaaacagagtacgtgtttgacgtggacaagaagcgttgcgttaagaaggaagaagcctcaggtctggtcctctcgggagaactgaccaaccctccctatcatgagctagctctggagggactgaagacccgacctgcggtcccgtacaaggtcgaaacaataggagtgataggcacaccggggtcgggcaagtcagctattatcaagtcaactgtcacggcacgagatcttgttaccagcggaaagaaagaaaattgtcgcgaaattgaggccgacgtgctaagactgaggggtatgcagattacgtcgaagacagtagattcggttatgctcaacggatgccacaaagccgtagaagtgctgtacgttgacgaagcgttcgcgtgccacgcaggagcactacttgccttgattgctatcgtcaggccccgcaagaaggtagtactatgcggagaccccatgcaatgcggattcttcaacatgatgcaactaaaggtacatttcaatcaccctgaaaaagacatatgcaccaagacattctacaagtatatctcccggcgttgcacacagccagttacagctattgtatcgacactgcattacgatggaaagatgaaaaccacgaacccgtgcaagaagaacattgaaatcgatattacaggggccacaaagccgaagccaggggatatcatcctgacatgtttccgcgggtgggttaagcaattgcaaatcgactatcccggacatgaagtaatgacagccgcggcctcacaagggctaaccagaaaaggagtgtatgccgtccggcaaaaagtcaatgaaaacccactgtacgcgatcacatcagagcatgtgaacgtgttgctcacccgcactgaggacaggctagtgtggaaaaccttgcagggcgacccatggattaagcagcccactaacatacctaaaggaaactttcaggctactatagaggactgggaagctgaacacaagggaataattgctgcaataaacagccccactccccgtgccaatccgttcagctgcaagaccaacgtttgctgggcgaaagcattggaaccgatactagccacggccggtatcgtacttaccggttgccagtggagcgaactgttcccacagtttgcggatgacaaaccacattcggccatttacgccttagacgtaatttgcattaagtttttcggcatggacttgacaagcggactgttttctaaacagagcatcccactaacgtaccatcccgccgattcagcgaggccggtagctcattgggacaacagcccaggaacccgcaagtatgggtacgatcacgccattgccgccgaactctcccgtagatttccggtgttccagctagctgggaagggcacacaacttgatttgcagacggggagaaccagagttatctctgcacagcataacctggtcccggtgaaccgcaatcttcctcacgccttagtccccgagtacaaggagaagcaacccggcccggtcaaaaaattcttgaaccagttcaaacaccactcagtacttgtggtatcagaggaaaaaattgaagctccccgtaagagaatcgaatggatcgccccgattggcatagccggtgcagataagaactacaacctggctttcgggtttccgccgcaggcacggtacgacctggtgttcatcaacattggaactaaatacagaaaccaccactttcagcagtgcgaagaccatgcggcgaccttaaaaaccctttcgcgttcggccctgaattgccttaacccaggaggcaccctcgtggtgaagtcctatggctacgccgaccgcaacagtgaggacgtagtcaccgctcttgccagaaagtttgtcagggtgtctgcagcgagaccagattgtgtctcaagcaatacagaaatgtacctgattttccgacaactagacaacagccgtacacggcaattcaccccgcaccatctgaattgcgtgatttcgtccgtgtatgagggtacaagagatggagttggagccgcgccgtcataccgcaccaaaagggagaatattgctgactgtcaagaggaagcagttgtcaacgcagccaatccgctgggtagaccaggcgaaggagtctgccgtgccatctataaacgttggccgaccagttttaccgattcagccacggagacaggcaccgcaagaatgactgtgtgcctaggaaagaaagtgatccacgcggtcggccctgatttccggaagcacccagaagcagaagccttgaaattgctacaaaacgcctaccatgcagtggcagacttagtaaatgaacataacatcaagtctgtcgccattccactgctatctacaggcatttacgcagccggaaaagaccgccttgaagtatcacttaactgcttgacaaccgcgctagacagaactgacgcggacgtaaccatctattgcctggataagaagtggaaggaaagaatcgacgcggcactccaacttaaggagtctgtaacagagctgaaggatgaagatatggagatcgacgatgagttagtatggattcatccagacagttgcttgaagggaagaaagggattcagtactacaaaaggaaaattgtattcgtacttcgaaggcaccaaattccatcaagcagcaaaagacatggcggagataaaggtcctgttccctaatgaccaggaaagtaatgaacaactgtgtgcctacatattgggtgagaccatggaagcaatccgcgaaaagtgcccggtcgaccataacccgtcgtctagcccgcccaaaacgttgccgtgcctttgcatgtatgccatgacgccagaaagggtccacagacttagaagcaataacgtcaaagaagttacagtatgctcctccaccccccttcctaagcacaaaattaagaatgttcagaaggttcagtgcacgaaagtagtcctgtttaatccgcacactcccgcattcgttcccgcccgtaagtacatagaagtgccagaacagcctaccgctcctcctgcacaggccgaggaggcccccgaagttgtagcgacaccgtcaccatctacagctgataacacctcgcttgatgtcacagacatctcactggatatggatgacagtagcgaaggctcacttttttcgagctttagcggatcggacaactctattactagtatggacagttggtcgtcaggacctagttcactagagatagtagaccgaaggcaggtggtggtggctgacgttcatgccgtccaagagcctgcccctattccaccgccaaggctaaagaagatggcccgcctggcagcggcaagaaaagagcccactccaccggcaagcaatagctctgagtccctccacctctcttttggtggggtatccatgtccctcggatcaattttcgacggagagacggcccgccaggcagcggtacaacccctggcaacaggccccacggatgtgcctatgtctttcggatcgttttccgacggagagattgatgagctgagccgcagagtaactgagtccgaacccgtcctgtttggatcatttgaaccgggcgaagtgaactcaattatatcgtcccgatcagccgtatcttttccactacgcaagcagagacgtagacgcaggagcaggaggactgaatactgactaaccggggtaggtgggtacatattttcgacggacacaggccctgggcacttgcaaaagaagtccgttctgcagaaccagcttacagaaccgaccttggagcgcaatgtcctggaaagaattcatgccccggtgctcgacacgtcgaaagaggaacaactcaaactcaggtaccagatgatgcccaccgaagccaacaaaagtaggtaccagtctcgtaaagtagaaaatcagaaagccataaccactgagcgactactgtcaggactacgactgtataactctgccacagatcagccagaatgctataagatcacctatccgaaaccattgtactccagtagcgtaccggcgaactactccgatccacagttcgctgtagctgtctgtaacaactatctgcatgagaactatccgacagtagcatcttatcagattactgacgagtacgatgcttacttggatatggtagacgggacagtcgcctgcctggatactgcaaccttctgccccgctaagcttagaagttacccgaaaaaacatgagtatagagccccgaatatccgcagtgcggttccatcagcgatgcagaacacgctacaaaatgtgctcattgccgcaactaaaagaaattgcaacgtcacgcagatgcgtgaactgccaacactggactcagcgacattcaatgtcgaatgctttcgaaaatatgcatgtaatgacgagtattgggaggagttcgctcggaagccaattaggattaccactgagtttgtcaccgcatatgtagctagactgaaaggccctaaggccgccgcactatttgcaaagacgtataatttggtcccattgcaagaagtgcctatggatagattcgtcatggacatgaaaagagacgtgaaagttacaccaggcacgaaacacacagaagaaagaccgaaagtacaagtgatacaagccgcagaacccctggcgactgcttacttatgcgggattcaccgggaattagtgcgtaggcttacggccgtcttgcttccaaacattcacacgctttttgacatgtcggcggaggattttgatgcaatcatagcagaacacttcaagcaaggcgacccggtactggagacggatatcgcatcattcgacaaaagccaagacgacgctatggcgttaaccggtctgatgatcttggaggacctgggtgtggatcaaccactactcgacttgatcgagtgcgcctttggagaaatatcatccacccatctacctacgggtactcgttttaaattcggggcgatgatgaaatccggaatgttcctcacactttttgtcaacacagttttgaatgtcgttatcgccagcagagtactagaagagcggcttaaaacgtccagatgtgcagcgttcattggcgacgacaacatcatacatggagtagtatctgacaaagaaatggctgagaggtgcgccacctggctcaacatggaggttaagatcatcgacgcagtcatcggtgagagaccaccttacttctgcggcggatttatcttgcaagattcggttacttccacagcgtgccgcgtggcggatcccctgaaaaggctgtttaagttgggtaaaccgctcccagccgacgacgagcaagacgaagacagaagacgcgctctgctagatgaaacaaaggcgtggtttagagtaggtataacaggcactttagcagtggccgtgacgacccggtatgaggtagacaatattacacctgtcctactggcattgagaacttttgcccagagcaaaagagcattccaagccatcagaggggaaataaagcatctctacggtggtcctaaatagtcagcatagtacatttcatctgactaatactacaacaccaccacctctagaacaaattcagctaccataatgatgcagagaggcaattttaggaaccaaagaaagattgttaagtgtttcaattgtggcaaagaagggcacacagccagaaattgcagggcccctaggaaaaagggctgttggaaatgtggaaaggaaggacaccaaatgaaagattgtactgagagacaggctaattttttagggaagatctggccttcctacaagggaaggccagggaattttcttcagagcagaccagagccaacagccccaccagaagagagcttcaggtctggggtagagacaacaactccccctcagaagcaggagccgatagacaaggaactgtatcctttaacttccctcaggtcactctttggcaacgacccctcgtcacaataaagataggggggcaactaaaggaagctctaatataaacaggagcagataatacaatattagaagaaatgagtttgccaggaagatggaaaccaaaaatactagtgggagttggaggttttatgaaagtaagacagtatgatcagatactcatagaaatctgtggacataaagctatatctacagtagtagtaggacctacacctgccaacgtaattggaagagatctgatgactcagattggttgcactttaaattttcccattagccctattgagactgtaccagtaaaattaaagccaggaatggatggcccaaaagttaaacaatggccattgacagaagaaaaaataaaagcattagtagaaatttgtacagagttggaaaaggaagggaaaatttcaaaaattgggcctgaaaatccatacaatactccagtatttgccataaagagaaaaaacagttcttcctccagatggagaaaagtagtagatctcagagaacttaataagagaactcaagacttctgggaagttcaattaggaataccacatcccgcagggatagaaaagaacaaatcagcaacaatactgtaagtgggtgatgcattttattcagttcccttagatgaagacttcaggaagtatactgcatttaccatacctagtataaacaatgagacaccagggattagatatcagtacaatgtgcttccaatgggatggaaaggatcaccagcaatattccaaagtagcatgacaaaaatcttagagccttttagaaaacaaaatccagacatagttatctgtcaatacgtggatgatttgttagtagcatctgacttagaaatagggcagcatagaacaaaaatagaggagctgagacaacatctgtggaggtggggactttacacaccagaccaaaaacatcagaaagaacatccattcctttggctgggttatgaactccatcctgataaatggacagtacagcctatagtgctgccagaaaaagacagctggactgtcaatgacatacagaagttagtggggaaattgaattgggcaagtcagatttacccagggattaaagtaaggcaattatgtaaactccttagaggaaccaaagcactaacagaagtaataccactaacagaagaagcagagctagaactggcagaaaacagagagattctaaaagaaccagtacatggagtgtattatgacccatcaaaagacttaatagcagaaatacagaagcaggggcaaggccaatggacatatcaaatttatcaagagccatttaaaaatctgaaaacaggaaaatatgcaagaatgaggggtgcccacactaatgatgtaaaacaattaacagaggcagtgcaaaaaataaccacagaaagcatagtaatatggggaaagactcctaaatttaaactgcccatacaaaaggaaacatgggaaacatggtggacagagtattggcaagccacctggattcctgagtgggagtttgttaatacccctcccttagtgaaattatggtaccagttagagaaagaacccatagtaggagcagaaaccttctatgtagatggggcagctaacagggagactaaattaggaaaagcaggatatgttactaatagaggaagacaaaaagttgtcaccctaactgacacaacaaatcagaagactgagttacaagcaatttatctagctttgcaggattcgggattagaagtaaacatagtaacagactcacaatatgcattaggaatcattcaagcacaaccagatcaaagtgaatcagagttagtcaatcaaataatagagcagttaataaaaaaggaaaaggtctatctggcatgggtaccagcacacaaaggaattggaggaaatgaacaagtagataaattagtcagtgctggaatcaggaaagtactatttttagatggaatagataaggcccaagatgaacatgagaaatatcacagtaattggagagcaatggctagtgattttaacctgccacctgtagtagcaaaagaaatagtagccagctgtgataaatgtcagctaaaaggagaagccatgcatggacaagtagactgtagtccaggaatatggcaactagattgtatacatttagaaggaaaagttatcatggtagcagttcatgtagccagtggatatatagaagcagaagttattccagcacaaacagggcaggaagcagcatattttcttttaaaattagcaggaagatggccagtaaaaacaatacatactgacaatggcagcaatttcaccggtgctacggttagggccgcctgttggtgggcgggaatcaagcaggcattttcaattccccgcaatccccaaagtcacggagtagtataatctatgcataaagaattaaagaaaattataggacaggtaagagatcaggctgaacatcttaagacagcagtacaaatggcagtattcatccacaattttaaaagaaaaggggggattggggggtacagtgcaggggaaagaatagtagacataatagcaacagacatacaaactaaagaattacaaaaacaaattacaaaaattcaaaattttcgggtttattacagggacagcagaaatccactttggaaaggaccagcaaagctcctctggaaaggtgaaggggcagtagtaatacaagataatagtgacataaaagtagtgccaagaagaaaagcaaagatcattagggattatggaaaacagatggcaggtgatgattgtgtggcaagtagacaggatgaggattagaacatggaaaagtttagtaaaacaccatatgtatgtttcagggaaagctaggggatggttttatagacatcactatgaaagccctcatccaagaataagttcagaagtacacatcccactaggggatgctagattggtaataacaacatattggggtctgcatacaggagaaagagactggcatttgggtcagggagtctccatagaatggaggaaaaagagatatagcacacaagtagaccctgaactagcagaccaactaattcatctgtattactttgactgtttttcagactctgctatggcgcgccacgtgacgcgtgcatgcatttaaatatcgagggcaggagcgagagggccaaggccagggagggcggccaccaccatcaccaccatcaccattagtaatgaggtaaccgtggggcccaatgatccgaccagcaaaactcgatgtacttccgaggaactgatgtgcataatgcatcaggctggtacattagatccccgcttaccgcgggcaatatagcaacactaaaaactcgatgtacttccgaggaagcgcagtgcataatgctgcgcagtgttgccacataaccactatattaaccatttatctagcggacgccaaaaactcaatgtatttctgaggaagcgtggtgcataatgccacgcagcgtctgcataacttttattatttcttttattaatcaacaaaattttgtttttaacatttcaaaaaaaaaaaaaaaaaaaaaaaaaaaaaaaaaaaaagggaattcctcgattaattaagcggccgc

SEQ ID NO: 12 - DNA, 11649 bp, Artificial Sequence
  Description of Artificial Sequence: Synthetic polynucleotide
  MISC_FEATURE (1)..(7646): Sindbis gene sequence
  MISC_FEATURE (7647)..(11160): Wild-type HIV-1 insert sequence
  MISC_FEATURE (11161)..(11649): Sindbis gene sequence
attgacggcgtagtacacactattgaatcaaacagccgaccaattgcactaccatcacaatggagaagccagtagtaaacgtagacgtagacccccagagtccgtttgtcgtgcaactgcaaaaaagcttcccgcaatttgaggtagtagcacagcaggtcactccaaatgaccatgctaatgccagagcattttcgcatctggccagtaaactaatcgagctggaggttcctaccacagcgacgatcttggacataggcagcgcaccggctcgtagaatgttttccgagcaccagtatcattgtgtctgccccatgcgtagtccagaagacccggaccgcatgatgaaatacgccagtaaactggcggaaaaagcgtgcaagattacaaacaagaacttgcatgagaagattaaggatctccggaccgtacttgatacgccggatgctgaaacaccatcgctctgctttcacaacgatgttacctgcaacatgcgtgccgaatattccgtcatgcaggacgtgtatatcaacgctcccggaactatctatcatcaggctatgaaaggcgtgcggaccctgtactggattggcttcgacaccacccagttcatgttctcggctatggcaggttcgtaccctgcgtacaacaccaactgggccgacgagaaagtccttgaagcgcgtaacatcggactttgcagcacaaagctgagtgaaggtaggacaggaaaattgtcgataatgaggaagaaggagttgaagcccgggtcgcgggtttatttctccgtaggatcgacactttatccagaacacagagccagcttgcagagctggcatcttccatcggtgttccacttgaatggaaagcagtcgtacacttgccgctgtgatacagtggtgagttgcgaaggctacgtagtgaagaaaatcaccatcagtcccgggatcacgggagaaaccgtgggatacgcggttacacacaatagcgagggcttcttgctatgcaaagttactgacacagtaaaaggagaacgggtatcgttccctgtgtgcacgtacatcccggccaccatatgcgatcagatgactggtataatggccacggatatatcacctgacgatgcacaaaaacttctggttgggctcaaccagcgaattgtcattaacggtaggactaacaggaacaccaacaccatgcaaaattaccttctgccgatcatagcacaagggttcagcaaatgggctaaggagcgcaaggatgatcttgataacgagaaaatgctgggtactagagaacgcaagcttacgtatggctgcttgtgggcgtttcgcactaagaaagtacattcgttttatcgcccacctggaacgcagacctgcgtaaaagtcccagcctcttttagcgcttttcccatgtcgtccgtatggacgacctctttgcccatgtcgctgaggcagaaattgaaactggcattgcaaccaaagaaggaggaaaaactgctgcaggtctcggaggaattagtcatggaggccaaggctgcttttgaggatgctcaggaggaagccagagcggagaagctccgagaagcacttccaccattagtggcagacaaaggcatcgaggcagccgcagaagttgtctgcgaagtggaggggctccaggcggacatcggagcagcattagttgaaaccccgcgcggtcacgtaaggataatacctcaagcaaatgaccgtatgatcggacagtatatcgttgtctcgccaaactctgtgctgaagaatgccaaactcgcaccagcgcacccgctagcagatcaggttaagatcataacacactccggaagatcaggaaggtacgcggtcgaaccatacgacgctaaagtactgatgccagcaggaggtgccgtaccatggccagaattcctagcactgagtgagagcgccacgttagtgtacaacgaaagagagtttgtgaaccgcaaactataccacattgccatgcatggccccgccaagaatacagaagaggagcagtacaaggttacaaaggcagagcttgcagaaacagagtacgtgtttgacgtggacaagaagcgttgcgttaagaaggaagaagcctcaggtctggtcctctcgggagaactgaccaaccctccctatcatgagctagctctggagggactgaagacccgacctgcggtcccgtacaaggtcgaaacaataggagtgataggcacaccggggtcgggcaagtcagctattatcaagtcaactgtcacggcacgagatcttgttaccagcggaaagaaagaaaattgtcgcgaaattgaggccgacgtgctaagactgaggggtatgcagattacgtcgaagacagtagattcggttatgctcaacggatgccacaaagccgtagaagtgctgtacgttgacgaagcgttcgcgtgccacgcaggagcactacttgccttgattgctatcgtcaggccccgcaagaaggtagtactatgcggagaccccatgcaatgcggattcttcaacatgatgcaactaaaggtacatttcaatcaccctgaaaaagacatatgcaccaagacattctacaagtatatctcccggcgttgcacacagccagttacagctattgtatcgacactgcattacgatggaaagatgaaaaccacgaacccgtgcaagaagaacattgaaatcgatattacaggggccacaaagccgaagccaggggatatcatcctgacatgtttccgcgggtgggttaagcaattgcaaatcgactatcccggacatgaagtaatgacagccgcggcctcacaagggctaaccagaaaaggagtgtatgccgtccggcaaaaagtcaatgaaaacccactgtacgcgatcacatcagagcatgtgaacgtgttgctcacccgcactgaggacaggctagtgtggaaaaccttgcagggcgacccatggattaagcagcccactaacatacctaaaggaaactttcaggctactatagaggactgggaagctgaacacaagggaataattgctgcaataaacagccccactccccgtgccaatccgttcagctgcaagaccaacgtttgctgggcgaaagcattggaaccgatactagccacggccggtatcgtacttaccggttgccagtggagcgaactgttcccacagtttgcggatgacaaaccacattcggccatttacgccttagacgtaatttgcattaagtttttcggcatggacttgacaagcggactgttttctaaacagagcatcccactaacgtaccatcccgccgattcagcgaggccggtagctcattgggacaacagcccaggaacccgcaagtatgggtacgatcacgccattgccgccgaactctcccgtagatttccggtgttccagctagctgggaagggcacacaacttgatttgcagacggggagaaccagagttatctctgcacagcataacctggtcccggtgaaccgcaatcttcctcacgccttagtccccgagtacaaggagaagcaacccggcccggtcaaaaaattcttgaaccagttcaaacaccactcagtacttgtggtatcagaggaaaaaattgaagctccccgtaagagaatcgaatggatcgccccgattggcatagccggtgcagataagaactacaacctggctttcgggtttccgccgcaggcacggtacgacctggtgttcatcaacattggaactaaatacagaaaccaccactttcagcagtgcgaagaccatgcggcgaccttaaaaaccctttcgcgttcggccctgaattgccttaacccaggaggcaccctcgtggtgaagtcctatggctacgccgaccgcaacagtgaggacgtagtcaccgctcttgccagaaagtttgtcagggtgtctgcagcgagaccagattgtgtctcaagcaatacagaaatgtacctgattttccgacaactagacaacagccgtacacggcaattcaccccgcaccatctgaattgcgtgatttcgtccgtgtatgagggtacaagagatggagttggagccgcgccgtcataccgcaccaaaagggagaatattgctgactgtcaagaggaagcagttgtcaacgcagccaatccgctgggtagaccaggcgaaggagtctgccgtgccatctataaacgttggccgaccagttttaccgattcagccacggagacaggcaccgcaagaatgactgtgtgcctaggaaagaaagtgatccacgcggtcggccctgatttccggaagcacccagaagcagaagccttgaaattgctacaaaacgcctaccatgcagtggcagacttagtaaatgaacataacatcaagtctgtcgccattccactgctatctacaggcatttacgcagccggaaaagaccgccttgaagtatcacttaactgcttgacaaccgcgctagacagaactgacgcggacgtaaccatctattgcctggataagaagtggaaggaaagaatcgacgcggcactccaacttaaggagtctgtaacagagctgaaggatgaagatatggagatcgacgatgagttagtatggattcatccagacagttgcttgaagggaagaaagggattcagtactacaaaaggaaaattgtattcgtacttcgaaggcaccaaattccatcaagcagcaaaagacatggcggagataaaggtcctgttccctaatgaccaggaaagtaatgaacaactgtgtgcctacatattgggtgagaccatggaagcaatccgcgaaaagtgcccggtcgaccataacccgtcgtctagcccgcccaaaacgttgccgtgcctttgcatgtatgccatgacgccagaaagggtccacagacttagaagcaataacgtcaaagaagttacagtatgctcctccaccccccttcctaagcacaaaattaagaatgttcagaaggttcagtgcacgaaagtagtcctgtttaatccgcacactcccgcattcgttcccgcccgtaagtacatagaagtgccagaacagcctaccgctcctcctgcacaggccgaggaggcccccgaagttgtagcgacaccgtcaccatctacagctgataacacctcgcttgatgtcacagacatctcactggatatggatgacagtagcgaaggctcacttttttcgagctttagcggatcggacaactctattactagtatggacagttggtcgtcaggacctagttcactagagatagtagaccgaaggcaggtggtggtggctgacgttcatgccgtccaagagcctgcccctattccaccgccaaggctaaagaagatggcccgcctggcagcggcaagaaaagagcccactccaccggcaagcaatagctctgagtccctccacctctcttttggtggggtatccatgtccctcggatcaattttcgacggagagacggcccgccaggcagcggtacaacccctggcaacaggccccacggatgtgcctatgtctttcggatcgttttccgacggagagattgatgagctgagccgcagagtaactgagtccgaacccgtcctgtttggatcatttgaaccgggcgaagtgaactcaattatatcgtcccgatcagccgtatcttttccactacgcaagcagagacgtagacgcaggagcaggaggactgaatactgactaaccggggtaggtgggtacatattttcgacggacacaggccctgggcacttgcaaaagaagtccgttctgcagaaccagcttacagaaccgaccttggagcgcaatgtcctggaaagaattcatgccccggtgctcgacacgtcgaaagaggaacaactcaaactcaggtaccagatgatgcccaccgaagccaacaaaagtaggtaccagtctcgtaaagtagaaaatcagaaagccataaccactgagcgactactgtcaggactacgactgtataactctgccacagatcagccagaatgctataagatcacctatccgaaaccattgtactccagtagcgtaccggcgaactactccgatccacagttcgctgtagctgtctgtaacaactatctgcatgagaactatccgacagtagcatcttatcagattactgacgagtacgatgcttacttggatatggtagacgggacagtcgcctgcctggatactgcaaccttctgccccgctaagcttagaagttacccgaaaaaacatgagtatagagccccgaatatccgcagtgcggttccatcagcgatgcagaacacgctacaaaatgtgctcattgccgcaactaaaagaaattgcaacgtcacgcagatgcgtgaactgccaacactggactcagcgacattcaatgtcgaatgctttcgaaaatatgcatgtaatgacgagtattgggaggagttcgctcggaagccaattaggattaccactgagtttgtcaccgcatatgtagctagactgaaaggccctaaggccgccgcactatttgcaaagacgtataatttggtcccattgcaagaagtgcctatggatagattcgtcatggacatgaaaagagacgtgaaagttacaccaggcacgaaacacacagaagaaagaccgaaagtacaagtgatacaagccgcagaacccctggcgactgcttacttatgcgggattcaccgggaattagtgcgtaggcttacggccgtcttgcttccaaacattcacacgctttttgacatgtcggcggaggattttgatgcaatcatagcagaacacttcaagcaaggcgacccggtactggagacggatatcgcatcattcgacaaaagccaagacgacgctatggcgttaaccggtctgatgatcttggaggacctgggtgtggatcaaccactactcgacttgatcgagtgcgcctttggagaaatatcatccacccatctacctacgggtactcgttttaaattcggggcgatgatgaaatccggaatgttcctcacactttttgtcaacacagttttgaatgtcgttatcgccagcagagtactagaagagcggcttaaaacgtccagatgtgcagcgttcattggcgacgacaacatcatacatggagtagtatctgacaaagaaatggctgagaggtgcgccacctggctcaacatggaggttaagatcatcgacgcagtcatcggtgagagaccaccttacttctgcggcggatttatcttgcaagattcggttacttccacagcgtgccgcgtggcggatcccctgaaaaggctgtttaagttgggtaaaccgctcccagccgacgacgagcaagacgaagacagaagacgcgctctgctagatgaaacaaaggcgtggtttagagtaggtataacaggcactttagcagtggccgtgacgacccggtatgaggtagacaatattacacctgtcctactggcattgagaacttttgcccagagcaaaagagcattccaagccatcagaggggaaataaagcatctctacggtggtcctaaatagtcagcatagtacatttcatctgactaatactacaacaccaccacctctagaacaaattcagctaccataatgatgcagagaggcaattttaggaaccaaagaaagattgttaagtgtttcaattgtggcaaagaagggcacacagccagaaattgcagggcccctaggaaaaagggctgttggaaatgtggaaaggaaggacaccaaatgaaagattgtactgagagacaggctaattttttagggaagatctggccttcctacaagggaaggccagggaattttcttcagagcagaccagagccaacagccccaccagaagagagcttcaggtctggggtagagacaacaactccccctcagaagcaggagccgatagacaaggaactgtatcctttaacttccctcaggtcactctttggcaacgacccctcgtcacaataaagataggggggcaactaaaggaagctctattataaacaggagcagatgatacagtattagaagaaatgagtttgccaggaagatggaaaccaaaaatgatagggggaattggaggttttatcaaagtaagacagtatgatcagatactcatagaaatctgtggacataaagctataggtacagtattagtaggacctacacctgtcaacataattggaagaaatctgttgactcagattggttgcactttaaattttcccattagccctattgagactgtaccagtaaaattaaagccaggaatggatggcccaaaagttaaacaatggccattgacagaagaaaaaataaaagcattagtagaaatttgtacagagatggaaaaggaagggaaaatttcaaaaattgggcctgaaaatccatacaatactccagtatttgccataaagaaaaaagacagtactaaatggagaaaattagtagatttcagagaacttaataagagaactcaagacttctgggaagttcaattaggaataccacatcccgcagggttaaaaaagaaaaaatcagtaacagtactgtaagtgggtgatgcatatttttcagttcccttagatgaagacttcaggaagtatactgcatttaccatacctagtataaacaatgagacaccagggattagatatcagtacaatgtgcttccacagggatggaaaggatcaccagcaatattccaaagtagcatgacaaaaatcttagagccttttagaaaacaaaatccagacatagttatctatcaatacatggatgatttgtatgtaggatctgacttagaaatagggcagcatagaacaaaaatagaggagctgagacaacatctgttgaggtggggacttaccacaccagacaaaaaacatcagaaagaacctccattcctttggatgggttatgaactccatcctgataaatggacagtacagcctatagtgctgccagaaaaagacagctggactgtcaatgacatacagaagttagtggggaaattgaattgggcaagtcagatttacccagggattaaagtaaggcaattatgtaaactccttagaggaaccaaagcactaacagaagtaataccactaacagaagaagcagagctagaactggcagaaaacagagagattctaaaagaaccagtacatggagtgtattatgacccatcaaaagacttaatagcagaaatacagaagcaggggcaaggccaatggacatatcaaatttatcaagagccatttaaaaatctgaaaacaggaaaatatgcaagaatgaggggtgcccacactaatgatgtaaaacaattaacagaggcagtgcaaaaaataaccacagaaagcatagtaatatggggaaagactcctaaatttaaactgcccatacaaaaggaaacatgggaaacatggtggacagagtattggcaagccacctggattcctgagtgggagtttgttaatacccctcccttagtgaaattatggtaccagttagagaaagaacccatagtaggagcagaaaccttctatgtagatggggcagctaacagggagactaaattaggaaaagcaggatatgttactaatagaggaagacaaaaagttgtcaccctaactgacacaacaaatcagaagactgagttacaagcaatttatctagctttgcaggattcgggattagaagtaaacatagtaacagactcacaatatgcattaggaatcattcaagcacaaccagatcaaagtgaatcagagttagtcaatcaaataatagagcagttaataaaaaaggaaaaggtctatctggcatgggtaccagcacacaaaggaattggaggaaatgaacaagtagataaattagtcagtgctggaatcaggaaagtactatttttagatggaatagataaggcccaagatgaacatgagaaatatcacagtaattggagagcaatggctagtgattttaacctgccacctgtagtagcaaaagaaatagtagccagctgtgataaatgtcagctaaaaggagaagccatgcatggacaagtagactgtagtccaggaatatggcaactagattgtacacatttagaaggaaaagttatcctggtagcagttcatgtagccagtggatatatagaagcagaagttattccagcagaaacagggcaggaaacagcatattttcttttaaaattagcaggaagatggccagtaaaaacaatacatactgacaatggcagcaatttcaccggtgctacggttagggccgcctgttggtgggcgggaatcaagcaggaatttggaattccctacaatccccaaagtcaaggagtagtataatctatgaataaagaattaaagaaaattataggacaggtaagagatcaggctgaacatcttaagacagcagtacaaatggcagtattcatccacaattttaaaagaaaaggggggattggggggtacagtgcaggggaaagaatagtagacataatagcaacagacatacaaactaaagaattacaaaaacaaattacaaaaattcaaaattttcgggtttattacagggacagcagaaatccactttggaaaggaccagcaaagctcctctggaaaggtgaaggggcagtagtaatacaagataatagtgacataaaagtagtgccaagaagaaaagcaaagatcattagggattatggaaaacagatggcaggtgatgattgtgtggcaagtagacaggatgaggattagaacatggaaaagtttagtaaaacaccatatgtatgtttcagggaaagctaggggatggttttatagacatcactatgaaagccctcatccaagaataagttcagaagtacacatcccactaggggatgctagattggtaataacaacatattggggtctgcatacaggagaaagagactggcatttgggtcagggagtctccatagaatggaggaaaaagagatatagcacacaagtagaccctgaactagcagaccaactaattcatctgtattactttgactgtttttcagactctgctatggcgcgccacgtgacgcgtgcatgcatttaaatatcgagggcaggagcgagagggccaaggccagggagggcggccaccaccatcaccaccatcaccattagtaatgaggtaaccgtggggcccaatgatccgaccagcaaaactcgatgtacttccgaggaactgatgtgcataatgcatcaggctggtacattagatccccgcttaccgcgggcaatatagcaacactaaaaactcgatgtacttccgaggaagcgcagtgcataatgctgcgcagtgttgccacataaccactatattaaccatttatctagcggacgccaaaaactcaatgtatttctgaggaagcgtggtgcataatgccacgcagcgtctgcataacttttattatttcttttattaatcaacaaaattttgtttttaacatttcaaaaaaaaaaaaaaaaaaaaaaaaaaaaaaaaaaaaagggaattcctcgattaattaagcggccgc

SEQ ID NO: 13 - DNA, 9675 bp, Artificial Sequence
  Description of Artificial Sequence: Synthetic polynucleotide
  MISC_FEATURE (1)..(7646): Sindbis gene sequence
  MISC_FEATURE (7647)..(9186): Mutant HIV-1 insert sequence
  MISC_FEATURE (9187)..(9675): Sindbis gene sequence
attgacggcgtagtacacactattgaatcaaacagccgaccaattgcactaccatcacaatggagaagccagtagtaaacgtagacgtagacccccagagtccgtttgtcgtgcaactgcaaaaaagcttcccgcaatttgaggtagtagcacagcaggtcactccaaatgaccatgctaatgccagagcattttcgcatctggccagtaaactaatcgagctggaggttcctaccacagcgacgatcttggacataggcagcgcaccggctcgtagaatgttttccgagcaccagtatcattgtgtctgccccatgcgtagtccagaagacccggaccgcatgatgaaatacgccagtaaactggcggaaaaagcgtgcaagattacaaacaagaacttgcatgagaagattaaggatctccggaccgtacttgatacgccggatgctgaaacaccatcgctctgctttcacaacgatgttacctgcaacatgcgtgccgaatattccgtcatgcaggacgtgtatatcaacgctcccggaactatctatcatcaggctatgaaaggcgtgcggaccctgtactggattggcttcgacaccacccagttcatgttctcggctatggcaggttcgtaccctgcgtacaacaccaactgggccgacgagaaagtccttgaagcgcgtaacatcggactttgcagcacaaagctgagtgaaggtaggacaggaaaattgtcgataatgaggaagaaggagttgaagcccgggtcgcgggtttatttctccgtaggatcgacactttatccagaacacagagccagcttgcagagctggcatcttccatcggtgttccacttgaatggaaagcagtcgtacacttgccgctgtgatacagtggtgagttgcgaaggctacgtagtgaagaaaatcaccatcagtcccgggatcacgggagaaaccgtgggatacgcggttacacacaatagcgagggcttcttgctatgcaaagttactgacacagtaaaaggagaacgggtatcgttccctgtgtgcacgtacatcccggccaccatatgcgatcagatgactggtataatggccacggatatatcacctgacgatgcacaaaaacttctggttgggctcaaccagcgaattgtcattaacggtaggactaacaggaacaccaacaccatgcaaaattaccttctgccgatcatagcacaagggttcagcaaatgggctaaggagcgcaaggatgatcttgataacgagaaaatgctgggtactagagaacgcaagcttacgtatggctgcttgtgggcgtttcgcactaagaaagtacattcgttttatcgcccacctggaacgcagacctgcgtaaaagtcccagcctcttttagcgcttttcccatgtcgtccgtatggacgacctctttgcccatgtcgctgaggcagaaattgaaactggcattgcaaccaaagaaggaggaaaaactgctgcaggtctcggaggaattagtcatggaggccaaggctgcttttgaggatgctcaggaggaagccagagcggagaagctccgagaagcacttccaccattagtggcagacaaaggcatcgaggcagccgcagaagttgtctgcgaagtggaggggctccaggcggacatcggagcagcattagttgaaaccccgcgcggtcacgtaaggataatacctcaagcaaatgaccgtatgatcggacagtatatcgttgtctcgccaaactctgtgctgaagaatgccaaactcgcaccagcgcacccgctagcagatcaggttaagatcataacacactccggaagatcaggaaggtacgcggtcgaaccatacgacgctaaagtactgatgccagcaggaggtgccgtaccatggccagaattcctagcactgagtgagagcgccacgttagtgtacaacgaaagagagtttgtgaaccgcaaactataccacattgccatgcatggccccgccaagaatacagaagaggagcagtacaaggttacaaaggcagagcttgcagaaacagagtacgtgtttgacgtggacaagaagcgttgcgttaagaaggaagaagcctcaggtctggtcctctcgggagaactgaccaaccctccctatcatgagctagctctggagggactgaagacccgacctgcggtcccgtacaaggtcgaaacaataggagtgataggcacaccggggtcgggcaagtcagctattatcaagtcaactgtcacggcacgagatcttgttaccagcggaaagaaagaaaattgtcgcgaaattgaggccgacgtgctaagactgaggggtatgcagattacgtcgaagacagtagattcggttatgctcaacggatgccacaaagccgtagaagtgctgtacgttgacgaagcgttcgcgtgccacgcaggagcactacttgccttgattgctatcgtcaggccccgcaagaaggtagtactatgcggagaccccatgcaatgcggattcttcaacatgatgcaactaaaggtacatttcaatcaccctgaaaaagacatatgcaccaagacattctacaagtatatctcccggcgttgcacacagccagttacagctattgtatcgacactgcattacgatggaaagatgaaaaccacgaacccgtgcaagaagaacattgaaatcgatattacaggggccacaaagccgaagccaggggatatcatcctgacatgtttccgcgggtgggttaagcaattgcaaatcgactatcccggacatgaagtaatgacagccgcggcctcacaagggctaaccagaaaaggagtgtatgccgtccggcaaaaagtcaatgaaaacccactgtacgcgatcacatcagagcatgtgaacgtgttgctcacccgcactgaggacaggctagtgtggaaaaccttgcagggcgacccatggattaagcagcccactaacatacctaaaggaaactttcaggctactatagaggactgggaagctgaacacaagggaataattgctgcaataaacagccccactccccgtgccaatccgttcagctgcaagaccaacgtttgctgggcgaaagcattggaaccgatactagccacggccggtatcgtacttaccggttgccagtggagcgaactgttcccacagtttgcggatgacaaaccacattcggccatttacgccttagacgtaatttgcattaagtttttcggcatggacttgacaagcggactgttttctaaacagagcatcccactaacgtaccatcccgccgattcagcgaggccggtagctcattgggacaacagcccaggaacccgcaagtatgggtacgatcacgccattgccgccgaactctcccgtagatttccggtgttccagctagctgggaagggcacacaacttgatttgcagacggggagaaccagagttatctctgcacagcataacctggtcccggtgaaccgcaatcttcctcacgccttagtccccgagtacaaggagaagcaacccggcccggtcaaaaaattcttgaaccagttcaaacaccactcagtacttgtggtatcagaggaaaaaattgaagctccccgtaagagaatcgaatggatcgccccgattggcatagccggtgcagataagaactacaacctggctttcgggtttccgccgcaggcacggtacgacctggtgttcatcaacattggaactaaatacagaaaccaccactttcagcagtgcgaagaccatgcggcgaccttaaaaaccctttcgcgttcggccctgaattgccttaacccaggaggcaccctcgtggtgaagtcctatggctacgccgaccgcaacagtgaggacgtagtcaccgctcttgccagaaagtttgtcagggtgtctgcagcgagaccagattgtgtctcaagcaatacagaaatgtacctgattttccgacaactagacaacagccgtacacggcaattcaccccgcaccatctgaattgcgtgatttcgtccgtgtatgagggtacaagagatggagttggagccgcgccgtcataccgcaccaaaagggagaatattgctgactgtcaagaggaagcagttgtcaacgcagccaatccgctgggtagaccaggcgaaggagtctgccgtgccatctataaacgttggccgaccagttttaccgattcagccacggagacaggcaccgcaagaatgactgtgtgcctaggaaagaaagtgatccacgcggtcggccctgatttccggaagcacccagaagcagaagccttgaaattgctacaaaacgcctaccatgcagtggcagacttagtaaatgaacataacatcaagtctgtcgccattccactgctatctacaggcatttacgcagccggaaaagaccgccttgaagtatcacttaactgcttgacaaccgcgctagacagaactgacgcggacgtaaccatctattgcctggataagaagtggaaggaaagaatcgacgcggcactccaacttaaggagtctgtaacagagctgaaggatgaagatatggagatcgacgatgagttagtatggattcatccagacagttgcttgaagggaagaaagggattcagtactacaaaaggaaaattgtattcgtacttcgaaggcaccaaattccatcaagcagcaaaagacatggcggagataaaggtcctgttccctaatgaccaggaaagtaatgaacaactgtgtgcctacatattgggtgagaccatggaagcaatccgcgaaaagtgcccggtcgaccataacccgtcgtctagcccgcccaaaacgttgccgtgcctttgcatgtatgccatgacgccagaaagggtccacagacttagaagcaataacgtcaaagaagttacagtatgctcctccaccccccttcctaagcacaaaattaagaatgttcagaaggttcagtgcacgaaagtagtcctgtttaatccgcacactcccgcattcgttcccgcccgtaagtacatagaagtgccagaacagcctaccgctcctcctgcacaggccgaggaggcccccgaagttgtagcgacaccgtcaccatctacagctgataacacctcgcttgatgtcacagacatctcactggatatggatgacagtagcgaaggctcacttttttcgagctttagcggatcggacaactctattactagtatggacagttggtcgtcaggacctagttcactagagatagtagaccgaaggcaggtggtggtggctgacgttcatgccgtccaagagcctgcccctattccaccgccaaggctaaagaagatggcccgcctggcagcggcaagaaaagagcccactccaccggcaagcaatagctctgagtccctccacctctcttttggtggggtatccatgtccctcggatcaattttcgacggagagacggcccgccaggcagcggtacaacccctggcaacaggccccacggatgtgcctatgtctttcggatcgttttccgacggagagattgatgagctgagccgcagagtaactgagtccgaacccgtcctgtttggatcatttgaaccgggcgaagtgaactcaattatatcgtcccgatcagccgtatcttttccactacgcaagcagagacgtagacgcaggagcaggaggactgaatactgactaaccggggtaggtgggtacatattttcgacggacacaggccctgggcacttgcaaaagaagtccgttctgcagaaccagcttacagaaccgaccttggagcgcaatgtcctggaaagaattcatgccccggtgctcgacacgtcgaaagaggaacaactcaaactcaggtaccagatgatgcccaccgaagccaacaaaagtaggtaccagtctcgtaaagtagaaaatcagaaagccataaccactgagcgactactgtcaggactacgactgtataactctgccacagatcagccagaatgctataagatcacctatccgaaaccattgtactccagtagcgtaccggcgaactactccgatccacagttcgctgtagctgtctgtaacaactatctgcatgagaactatccgacagtagcatcttatcagattactgacgagtacgatgcttacttggatatggtagacgggacagtcgcctgcctggatactgcaaccttctgccccgctaagcttagaagttacccgaaaaaacatgagtatagagccccgaatatccgcagtgcggttccatcagcgatgcagaacacgctacaaaatgtgctcattgccgcaactaaaagaaattgcaacgtcacgcagatgcgtgaactgccaacactggactcagcgacattcaatgtcgaatgctttcgaaaatatgcatgtaatgacgagtattgggaggagttcgctcggaagccaattaggattaccactgagtttgtcaccgcatatgtagctagactgaaaggccctaaggccgccgcactatttgcaaagacgtataatttggtcccattgcaagaagtgcctatggatagattcgtcatggacatgaaaagagacgtgaaagttacaccaggcacgaaacacacagaagaaagaccgaaagtacaagtgatacaagccgcagaacccctggcgactgcttacttatgcgggattcaccgggaattagtgcgtaggcttacggccgtcttgcttccaaacattcacacgctttttgacatgtcggcggaggattttgatgcaatcatagcagaacacttcaagcaaggcgacccggtactggagacggatatcgcatcattcgacaaaagccaagacgacgctatggcgttaaccggtctgatgatcttggaggacctgggtgtggatcaaccactactcgacttgatcgagtgcgcctttggagaaatatcatccacccatctacctacgggtactcgttttaaattcggggcgatgatgaaatccggaatgttcctcacactttttgtcaacacagttttgaatgtcgttatcgccagcagagtactagaagagcggcttaaaacgtccagatgtgcagcgttcattggcgacgacaacatcatacatggagtagtatctgacaaagaaatggctgagaggtgcgccacctggctcaacatggaggttaagatcatcgacgcagtcatcggtgagagaccaccttacttctgcggcggatttatcttgcaagattcggttacttccacagcgtgccgcgtggcggatcccctgaaaaggctgtttaagttgggtaaaccgctcccagccgacgacgagcaagacgaagacagaagacgcgctctgctagatgaaacaaaggcgtggtttagagtaggtataacaggcactttagcagtggccgtgacgacccggtatgaggtagacaatattacacctgtcctactggcattgagaacttttgcccagagcaaaagagcattccaagccatcagaggggaaataaagcatctctacggtggtcctaaatagtcagcatagtacatttcatctgactaatactacaacaccaccacctctagaatgatctgtagtgctacagaaaaattgtgggtcacagtctattatggggtacctgtgtggaaggaagcaaccaccactctattttgtgcatcagatgctaaagcatatgatacagaggtacataatgtttgggccacacatgcctgtgtacccacagaccccaacccacaagaagtagtattggtaaatgtgacagaaaattttaacatgtggaaaaatgacatggtagaacagatgcatgaggatataatcagtttatgggatcaaagcctaaagccatgtgtaaaattaaccccactctgtgttagtttaaagtgcactgatttgaagaatgatactaataccaatagtagtagcgggagaatgataatggagaaaggagagataaaaaactgctctttcaatatcagcacaagcataagaggtaaggtgcagaaagaatatgcatttttttataaacttgatataataccaatagataatgatactaccagctataagttgacaagttgtaacacctcagtcattacacaggcctgtccaaaggtatcctttgagccaattcccatacattattgtgccccggctggttttgcgattctaaaatgtaataataagacgttcaatggaacaggaccatgtacaaatgtcagcacagtacaatgtacacatggaattaggccagtagtatcaactcaactgctgttaaatggcagtctagcagaagaagaggtagtaattagatctgtcaatttcacggacaatgctaaaaccataatagtacagctgaacacatctgtagaaattaattgtacaagacccaacaacaatacaagaaaaagaatccgtatccagagaggaccagggagagcatttgttacaataggaaaaataggaaatatgagacaagcacattgtaacattagtagagcaaaatggaataacactttaaaacagatagctagcaaattaagagaacaatttggaaataataaaacaataatctttaagcaatcctcaggaggggacccagaaattgtaacgcacagttttaattgtggaggggaatttttctactgtaattcaacacaactgtttaatagtacttggtttaatagtacttggagtactgaagggtcaaataacactgaaggaagtgacacaatcaccctcccatgcagaataaaacaaattataaacatgtggcagaaagtaggaaaagcaatgtatgcccctcccatcagtggacaaattagatgttcatcaaatattacagggctgctattaacaagagatggtggtaatagcaacaatgagtccgagatcttcagacctggaggaggagatatgagggacaattggagaagtgaattatataaatataaagtagtaaaaattgaaccattaggagtagcacccaccaaggcaaagagaagagtggtgcagagagaaaaaagagcagtgggaataggagctttgttccttgggttcttgggagcagcaggaagcactatgggcgcagcctcggcgcgccacgtgacgcgtgcatgcatttaaatatcgagggcaggagcgagagggccaaggccagggagggcggccaccaccatcaccaccatcaccattagtaatgaggtaaccgtggggcccaatgatccgaccagcaaaactcgatgtacttccgaggaactgatgtgcataatgcatcaggctggtacattagatccccgcttaccgcgggcaatatagcaacactaaaaactcgatgtacttccgaggaagcgcagtgcataatgctgcgcagtgttgccacataaccactatattaaccatttatctagcggacgccaaaaactcaatgtatttctgaggaagcgtggtgcataatgccacgcagcgtctgcataacttttattatttcttttattaatcaacaaaattttgtttttaacatttcaaaaaaaaaaaaaaaaaaaaaaaaaaaaaaaaaaaaagggaattcctcgattaattaagcggccgc

SEQ ID NO: 14 - DNA, 9670 bp, Artificial Sequence
  Description of Artificial Sequence: Synthetic polynucleotide
  MISC_FEATURE (1)..(7646): Sindbis gene sequence
  MISC_FEATURE (7647)..(9181): Wild-type HIV-1 insert sequence
  MISC_FEATURE (9182)..(9670): Sindbis gene sequence
attgacggcgtagtacacactattgaatcaaacagccgaccaattgcactaccatcacaatggagaagccagtagtaaacgtagacgtagacccccagagtccgtttgtcgtgcaactgcaaaaaagcttcccgcaatttgaggtagtagcacagcaggtcactccaaatgaccatgctaatgccagagcattttcgcatctggccagtaaactaatcgagctggaggttcctaccacagcgacgatcttggacataggcagcgcaccggctcgtagaatgttttccgagcaccagtatcattgtgtctgccccatgcgtagtccagaagacccggaccgcatgatgaaatacgccagtaaactggcggaaaaagcgtgcaagattacaaacaagaacttgcatgagaagattaaggatctccggaccgtacttgatacgccggatgctgaaacaccatcgctctgctttcacaacgatgttacctgcaacatgcgtgccgaatattccgtcatgcaggacgtgtatatcaacgctcccggaactatctatcatcaggctatgaaaggcgtgcggaccctgtactggattggcttcgacaccacccagttcatgttctcggctatggcaggttcgtaccctgcgtacaacaccaactgggccgacgagaaagtccttgaagcgcgtaacatcggactttgcagcacaaagctgagtgaaggtaggacaggaaaattgtcgataatgaggaagaaggagttgaagcccgggtcgcgggtttatttctccgtaggatcgacactttatccagaacacagagccagcttgcagagctggcatcttccatcggtgttccacttgaatggaaagcagtcgtacacttgccgctgtgatacagtggtgagttgcgaaggctacgtagtgaagaaaatcaccatcagtcccgggatcacgggagaaaccgtgggatacgcggttacacacaatagcgagggcttcttgctatgcaaagttactgacacagtaaaaggagaacgggtatcgttccctgtgtgcacgtacatcccggccaccatatgcgatcagatgactggtataatggccacggatatatcacctgacgatgcacaaaaacttctggttgggctcaaccagcgaattgtcattaacggtaggactaacaggaacaccaacaccatgcaaaattaccttctgccgatcatagcacaagggttcagcaaatgggctaaggagcgcaaggatgatcttgataacgagaaaatgctgggtactagagaacgcaagcttacgtatggctgcttgtgggcgtttcgcactaagaaagtacattcgttttatcgcccacctggaacgcagacctgcgtaaaagtcccagcctcttttagcgcttttcccatgtcgtccgtatggacgacctctttgcccatgtcgctgaggcagaaattgaaactggcattgcaaccaaagaaggaggaaaaactgctgcaggtctcggaggaattagtcatggaggccaaggctgcttttgaggatgctcaggaggaagccagagcggagaagctccgagaagcacttccaccattagtggcagacaaaggcatcgaggcagccgcagaagttgtctgcgaagtggaggggctccaggcggacatcggagcagcattagttgaaaccccgcgcggtcacgtaaggataatacctcaagcaaatgaccgtatgatcggacagtatatcgttgtctcgccaaactctgtgctgaagaatgccaaactcgcaccagcgcacccgctagcagatcaggttaagatcataacacactccggaagatcaggaaggtacgcggtcgaaccatacgacgctaaagtactgatgccagcaggaggtgccgtaccatggccagaattcctagcactgagtgagagcgccacgttagtgtacaacgaaagagagtttgtgaaccgcaaactataccacattgccatgcatggccccgccaagaatacagaagaggagcagtacaaggttacaaaggcagagcttgcagaaacagagtacgtgtttgacgtggacaagaagcgttgcgttaagaaggaagaagcctcaggtctggtcctctcgggagaactgaccaaccctccctatcatgagctagctctggagggactgaagacccgacctgcggtcccgtacaaggtcgaaacaataggagtgataggcacaccggggtcgggcaagtcagctattatcaagtcaactgtcacggcacgagatcttgttaccagcggaaagaaagaaaattgtcgcgaaattgaggccgacgtgctaagactgaggggtatgcagattacgtcgaagacagtagattcggttatgctcaacggatgccacaaagccgtagaagtgctgtacgttgacgaagcgttcgcgtgccacgcaggagcactacttgccttgattgctatcgtcaggccccgcaagaaggtagtactatgcggagaccccatgcaatgcggattcttcaacatgatgcaactaaaggtacatttcaatcaccctgaaaaagacatatgcaccaagacattctacaagtatatctcccggcgttgcacacagccagttacagctattgtatcgacactgcattacgatggaaagatgaaaaccacgaacccgtgcaagaagaacattgaaatcgatattacaggggccacaaagccgaagccaggggatatcatcctgacatgtttccgcgggtgggttaagcaattgcaaatcgactatcccggacatgaagtaatgacagccgcggcctcacaagggctaaccagaaaaggagtgtatgccgtccggcaaaaagtcaatgaaaacccactgtacgcgatcacatcagagcatgtgaacgtgttgctcacccgcactgaggacaggctagtgtggaaaaccttgcagggcgacccatggattaagcagcccactaacatacctaaaggaaactttcaggctactatagaggactgggaagctgaacacaagggaataattgctgcaataaacagccccactccccgtgccaatccgttcagctgcaagaccaacgtttgctgggcgaaagcattggaaccgatactagccacggccggtatcgtacttaccggttgccagtggagcgaactgttcccacagtttgcggatgacaaaccacattcggccatttacgccttagacgtaatttgcattaagtttttcggcatggacttgacaagcggactgttttctaaacagagcatcccactaacgtaccatcccgccgattcagcgaggccggtagctcattgggacaacagcccaggaacccgcaagtatgggtacgatcacgccattgccgccgaactctcccgtagatttccggtgttccagctagctgggaagggcacacaacttgatttgcagacggggagaaccagagttatctctgcacagcataacctggtcccggtgaaccgcaatcttcctcacgccttagtccccgagtacaaggagaagcaacccggcccggtcaaaaaattcttgaaccagttcaaacaccactcagtacttgtggtatcagaggaaaaaattgaagctccccgtaagagaatcgaatggatcgccccgattggcatagccggtgcagataagaactacaacctggctttcgggtttccgccgcaggcacggtacgacctggtgttcatcaacattggaactaaatacagaaaccaccactttcagcagtgcgaagaccatgcggcgaccttaaaaaccctttcgcgttcggccctgaattgccttaacccaggaggcaccctcgtggtgaagtcctatggctacgccgaccgcaacagtgaggacgtagtcaccgctcttgccagaaagtttgtcagggtgtctgcagcgagaccagattgtgtctcaagcaatacagaaatgtacctgattttccgacaactagacaacagccgtacacggcaattcaccccgcaccatctgaattgcgtgatttcgtccgtgtatgagggtacaagagatggagttggagccgcgccgtcataccgcaccaaaagggagaatattgctgactgtcaagaggaagcagttgtcaacgcagccaatccgctgggtagaccaggcgaaggagtctgccgtgccatctataaacgttggccgaccagttttaccgattcagccacggagacaggcaccgcaagaatgactgtgtgcctaggaaagaaagtgatccacgcggtcggccctgatttccggaagcacccagaagcagaagccttgaaattgctacaaaacgcctaccatgcagtggcagacttagtaaatgaacataacatcaagtctgtcgccattccactgctatctacaggcatttacgcagccggaaaagaccgccttgaagtatcacttaactgcttgacaaccgcgctagacagaactgacgcggacgtaaccatctattgcctggataagaagtggaaggaaagaatcgacgcggcactccaacttaaggagtctgtaacagagctgaaggatgaagatatggagatcgacgatgagttagtatggattcatccagacagttgcttgaagggaagaaagggattcagtactacaaaaggaaaattgtattcgtacttcgaaggcaccaaattccatcaagcagcaaaagacatggcggagataaaggtcctgttccctaatgaccaggaaagtaatgaacaactgtgtgcctacatattgggtgagaccatggaagcaatccgcgaaaagtgcccggtcgaccataacccgtcgtctagcccgcccaaaacgttgccgtgcctttgcatgtatgccatgacgccagaaagggtccacagacttagaagcaataacgtcaaagaagttacagtatgctcctccaccccccttcctaagcacaaaattaagaatgttcagaaggttcagtgcacgaaagtagtcctgtttaatccgcacactcccgcattcgttcccgcccgtaagtacatagaagtgccagaacagcctaccgctcctcctgcacaggccgaggaggcccccgaagttgtagcgacaccgtcaccatctacagctgataacacctcgcttgatgtcacagacatctcactggatatggatgacagtagcgaaggctcacttttttcgagctttagcggatcggacaactctattactagtatggacagttggtcgtcaggacctagttcactagagatagtagaccgaaggcaggtggtggtggctgacgttcatgccgtccaagagcctgcccctattccaccgccaaggctaaagaagatggcccgcctggcagcggcaagaaaagagcccactccaccggcaagcaatagctctgagtccctccacctctcttttggtggggtatccatgtccctcggatcaattttcgacggagagacggcccgccaggcagcggtacaacccctggcaacaggccccacggatgtgcctatgtctttcggatcgttttccgacggagagattgatgagctgagccgcagagtaactgagtccgaacccgtcctgtttggatcatttgaaccgggcgaagtgaactcaattatatcgtcccgatcagccgtatcttttccactacgcaagcagagacgtagacgcaggagcaggaggactgaatactgactaaccggggtaggtgggtacatattttcgacggacacaggccctgggcacttgcaaaagaagtccgttctgcagaaccagcttacagaaccgaccttggagcgcaatgtcctggaaagaattcatgccccggtgctcgacacgtcgaaagaggaacaactcaaactcaggtaccagatgatgcccaccgaagccaacaaaagtaggtaccagtctcgtaaagtagaaaatcagaaagccataaccactgagcgactactgtcaggactacgactgtataactctgccacagatcagccagaatgctataagatcacctatccgaaaccattgtactccagtagcgtaccggcgaactactccgatccacagttcgctgtagctgtctgtaacaactatctgcatgagaactatccgacagtagcatcttatcagattactgacgagtacgatgcttacttggatatggtagacgggacagtcgcctgcctggatactgcaaccttctgccccgctaagcttagaagttacccgaaaaaacatgagtatagagccccgaatatccgcagtgcggttccatcagcgatgcagaacacgctacaaaatgtgctcattgccgcaactaaaagaaattgcaacgtcacgcagatgcgtgaactgccaacactggactcagcgacattcaatgtcgaatgctttcgaaaatatgcatgtaatgacgagtattgggaggagttcgctcggaagccaattaggattaccactgagtttgtcaccgcatatgtagctagactgaaaggccctaaggccgccgcactatttgcaaagacgtataatttggtcccattgcaagaagtgcctatggatagattcgtcatggacatgaaaagagacgtgaaagttacaccaggcacgaaacacacagaagaaagaccgaaagtacaagtgatacaagccgcagaacccctggcgactgcttacttatgcgggattcaccgggaattagtgcgtaggcttacggccgtcttgcttccaaacattcacacgctttttgacatgtcggcggaggattttgatgcaatcatagcagaacacttcaagcaaggcgacccggtactggagacggatatcgcatcattcgacaaaagccaagacgacgctatggcgttaaccggtctgatgatcttggaggacctgggtgtggatcaaccactactcgacttgatcgagtgcgcctttggagaaatatcatccacccatctacctacgggtactcgttttaaattcggggcgatgatgaaatccggaatgttcctcacactttttgtcaacacagttttgaatgtcgttatcgccagcagagtactagaagagcggcttaaaacgtccagatgtgcagcgttcattggcgacgacaacatcatacatggagtagtatctgacaaagaaatggctgagaggtgcgccacctggctcaacatggaggttaagatcatcgacgcagtcatcggtgagagaccaccttacttctgcggcggatttatcttgcaagattcggttacttccacagcgtgccgcgtggcggatcccctgaaaaggctgtttaagttgggtaaaccgctcccagccgacgacgagcaagacgaagacagaagacgcgctctgctagatgaaacaaaggcgtggtttagagtaggtataacaggcactttagcagtggccgtgacgacccggtatgaggtagacaatattacacctgtcctactggcattgagaacttttgcccagagcaaaagagcattccaagccatcagaggggaaataaagcatctctacggtggtcctaaatagtcagcatagtacatttcatctgactaatactacaacaccaccacctctagaatgatctgtagtgctacagaaaaattgtgggtcacagtctattatggggtacctgtgtggaaagaagcaaccaccactctattttgtgcatcagatgctaaagcatatgatacagaggtacataatgtttgggccacacatgcctgtgtacccacagaccccaacccacaagaagtagaattggaaaatgtgacagaaaattttaacatgtggaaaaataacatggtagaacagatgcatgaggatataatcagtttatgggatcaaagcctaaagccatgtgtaaaattaactccactctgtgttactttaaattgcactgatttgaggaatgctactaatgggaatgacactaataccactagtagtagcagggaaatgatggggggaggagaaatgaaaaattgctctttcaaaatcaccacaaacataagaggtaaggtgcagaaagaatatgcacttttttataaacttgatatagtaccaatagataataatagtaataatagatataggttgataagttgtaacacctcagtcattacacaggcctgtccaaagatatcctttgagccaattcccatacattattgtgccccggctggttttgcgattctaaagtgtaaagataagaagttcaatggaaaaggaccatgttcaaatgtcagcacagtacaatgtacacatgggattaggccagtagtatcaactcaactgctgttaaatggcagtctagcagaagaagaggtagtaattagatccgaaaatttcgcggacaatgctaaaaccataatagtacagctgaatgaatctgtagaaattaattgtacaagacccaacaacaatacaagaaaaagtatacatataggaccaggcagagcattatatacaacaggaaaaataataggagatataagacaagcacattgtaaccttagtagagcaaaatggaatgacactttaaataaaatagttataaaattaagagaacaatttgggaataaaacaatagtctttaagcattcctcaggaggggacccagaaattgtgacgcacagttttaattgtggaggggaatttttctactgtaattcaacacaactgtttaatagtacttggaatgttactgaagagtcaaataacactgtagaaaataacacaatcacactcccatgcagaataaaacaaattataaacatgtggcagaaagtaggaagagcaatgtatgcccctcccatcagaggacaaattagatgttcatcaaatattacagggctgctattaacaagagatggtggtccagaggacaacaagaccgaggtcttcagacctggaggaggagatatgagggacaattggagaagtgaattatataaatataaagtagtaaaaattgaaccattaggagtagcacccaccaaggcaaagagaagagtggtgcagagagaaaaaagagcagtgggaataggagctgtgttccttgggttcttgggagcagcaggaagcactatgggcgcagctggcgcgccacgtgacgcgtgcatgcatttaaatatcgagggcaggagcgagagggccaaggccagggagggcggccaccaccatcaccaccatcaccattagtaatgaggtaaccgtggggcccaatgatccgaccagcaaaactcgatgtacttccgaggaactgatgtgcataatgcatcaggctggtacattagatccccgcttaccgcgggcaatatagcaacactaaaaactcgatgtacttccgaggaagcgcagtgcataatgctgcgcagtgttgccacataaccactatattaaccatttatctagcggacgccaaaaactcaatgtatttctgaggaagcgtggtgcataatgccacgcagcgtctgcataacttttattatttcttttattaatcaacaaaattttgtttttaacatttcaaaaaaaaaaaaaaaaaaaaaaaaaaaaaaaaaaaaagggaattcctcgattaattaagcggccgc

SEQ ID NO: 15 - DNA, 10272 bp, Zika virus
atgaaaaaccccaaagaagaaatccggaggatccggattgtcaatatgctaaaacgcggagtagcccgtgtgagcccctttgggggcttgaagaggctgccagccggacttctgctgggtcatgggcccatcaggatggtcttggcgatactagcctttttgagattcacggcaatcaagccatcactgggtctcatcaatagatggggttcagtggggaaaaaagaggctatggaaataataaagaagttcaagaaagatctggctgccatgctgagaataatcaatgctaggaaggagaagaagagacgaggcacagatactagtgtcggaattgttggcctcctgctgaccacagccatggcagtggaggtcactagacgtgggagtgcatactatatgtacttggacagaagcgatgctggggaggccatatcttttccaaccacactggggatgaacaagtgttacatacagatcatggatcttggacacatgtgtgatgccaccatgagctatgaatgccctatgttggatgagggggtagaaccagatgacgtcgattgttggtgcaacacgacatcaacttgggttgtgtacggaacctgccaccacaaaaaaggtgaagcacggagatctagaagagctgtgacgctcccctcccattccactaggaagctgcaaacgcggtcgcagacctggttggaatcaagagaatatacaaagcacctgattagagtcgaaaattggatattcaggaaccctggcttcgcgttagcagcagctgccatcgcctggcttttgggaagttcaacgagccaaaaagtcatatacttggtcatgatactgctgattgccccggcatacagcatcaggtgcataggagtcagcaatagggactttgtggaaggtatgtcaggtgggacttgggttgatgttgtcttggaacatggaggttgtgttaccgtaatggcacaggacaaaccggctgtcgacatagagctggttacaacaacagtcagcaacatggcggaggtaagatcctattgctatgaggcatcaatatcggacatggcttcggacagccgctgcccaacacaaggtgaagcctaccttgacaagcagtcagacactcaatatgtctgcaaaagaacgttagtggacagaggctggggaaatggatgtggactttttggcaaagggagcctggtgacatgcgctaagtttgcatgctccaagaaaatgaccgggaagagcatccagccagagaatctggagtaccggataatgctgtcagttcatggctcccagcacagtgggatgatcgttaatgacacaggacatgaaactgatgagaatagagcgaaggttgagataacgcccaattcaccaagagctgaagccaccctggggggttttggaagcctaggacttgattgtgaaccgaggacaggccttgacttttcagatttgtattacttgactatgaataacaagcactggttggttcacaaggagtggttccacgacattccattaccttggcatgctggggcagacaccggaactccacattggaacaacaaagaagcattggtagagttcaaggacgcacatgccaaaaggcaaactgtcgtggttctagggagtcaagaaggagcagttcacacggcccttgctggagctctggaggctgagatggatggtgcaaagggaaggctgtcctctggccacttgaaatgtcgcctgaaaatggataaacttagattgaagggcgtgtcatactccttgtgtaccgcagcgttcacattcaccaagatcccggctgaaacactgcacgggacagtcacagtggaggtacagtacgcagggacagatggaccctgcaaggttccagctcagatggcggtggacatgcaaactctgaccccagttgggaggctgataaccgctaaccctgtaatcactgaaagcactgagaactctaagatgatgctggaacttgatccaccatttggggactcttacattgtcataggagtcggggagaagaagatcacccatcactggcacaggagtggcagcaccattggaaaagcatttgaagccactgtgagaggtgccaagagaatggcagtcttgggagacacagcctgggattttggatcagttggaggtgctctcaactcattgggcaagggcatccatcaaatttttggagcagctttcaaatcattgtttggaggaatgtcctggttctcacaaattctcattggaacgttgctggtgtggttgggtctgaatacaaagaatggatctatttcccttacgtgcttggccttagggggagtgttgatctttttatccacagccgtctctgctgatgtggggtgctcggtggacttctcaaagaaggaaacgagatgcggtacgggggtgttcgtctataacgacgttgatgcctggagggacaggtacaagtaccatcctgactcccctcgtagattagcagcagcagtcaagcaagcctgggragatgggatctgtgggatctcctctgtttcaagaatggaaaacatcatgtggagatcagtagaaggggagctcaacgcaatcctggaagagaatggagttcaactgacggtcgttgtgggatctgtaaaaaaccccatgtggagaggtccacagagattgcccgtgcctgtgaacgagctgccccacggctggaaggcttgggggaaatcgtacttcgtcagagcagcaaagacaaataacagctttgtcgtggatggtgacacactgaaggaatgcccactcaaacatagagcatggaacagctttcttgtggaggatcatgggttcggggtatttcacactagtgtctggctcaaggttagagaagattattcattagagtgtgatccagccgttattggaacagctgctaagggaaaggaggctgtgcacagtgatctaggctactggattgagagtgagaagaatgacacatggaggctgaagagggcccacctgatcgagatgaaaacatgtgaatggccaaagtcccacacattgtggacagatggaatagaagaaagtgatctgatcatacccaagtctttagctgggccactcagccatcacaacaccagagagggctacaggactcaaatgaaagggccatggcacagtgaagagcttgaaattcggtttgaggaatgcccaggcactaaggtccacgtggaggaaacatgtggaacaagaggaccatctctgagatcaaccactgcaagcggaagggtgatcgaggaatggtgctgcagggaatgcacaatgcccccactgtcgttccgggctaaagatggctgttggtatggaatggagataaggcccaggaaagaaccagaaagtaacttagtaaggtcaatggtgactgcaggatcaactgatcacatggatcacttctcccttggagtgcttgtgattctgctcatggtgcaggaagggctgaagaagagaatgaccacaaagatcatcataagcacatcaatggcagtgctggtagctatgatcctgggaggattttcaatgagtgacctggccaagcttgcaattttgatgggtgccacctttgcggaaatgaacactggaggagatgtagctcatctggcgctgatagcggcattcaaagtcagacctgcgttgctggtatctttcatcttcagagctaattggacaccccgtgagagcatgctgctggccctggcttcgtgtcttctgcaaactgcgatctccgccttggaaggcgacctgatggttctcatcaatggttttgctttggcctggttggcaatacgagcgatggttgttccacgcactgacaacatcaccttggcaatcctgactgcgctgacaccactggcccggggcacgctgcttgtggcgtggagagcaggccttgctacttgcggggggttcatgcttctctctctgaaggggaagggcagtgtgaagaagaacctaccatttgtcatggccttgggactcaccgctgtgaggctggtcgaccccatcaacgtggtgggactgctgttgctcacaaggagtgggaagcggagctggccccctagtgaagtactcacagctgttggtctgatatgcgcgttggccggagggttcgccaaggcggatatagagatggctgggcccatggccgcggtcggtctgctaattgtcagttacgtggtctcaggaaagagtgtggacatgtacattgaaagagcaggtgacatcacatgggaaaaagatgcggaagtcactggaaacagtccccggctcgatgtggcactggatgagagtggtgatttctccctagtggaggatgatggtccccccatgagagagatcatactcaaagtggtcctgatgaccatctgtggcatgaacccaatagccataccctttgcagctggagcgtggtacgtgtatgtgaagactggaaaaaggagtggtgctctatgggatgtgcctgctcccaaggaagtaaaaaagggggagaccacagatggagtgtacagagtaatgactcgtagactgcttggttcaacacaagttggagtgggagtcatgcaagagggggtcttccacactatgtggcacgtcacaaaaggatccgcgctgagaagcggtgaagggagacttgatccatactggggagatgtcaagcaggatctggtgtcatattgtggtccgtggaagctagacgccgcctgggacgggcacagcgaggtgcagctcttggccgtgccccccggagagagagcgaggaacatccagactccgcccggaatatttaagacaaaggatggggacattggagcagttgcgttggactacccagcaggaacttcaggatctccaatcctagacaagtgtgggagagtgataggactctatggtaatggggtcgtgataaaaaatgggagttatgttagtgccatcacccaagggaggagggaggaagagactcctgttgagtgcttcgagccttcgatgttgaagaagaagcagctaactgtcttagacctgcatcctggagctgggaaaaccaggagagttcttcctgaaatagtccgtgaagccataaaaacaagactccgtactgtgatcttagctccaaccagggttgtcgctgctgaaatggaggaagcccttagagggcttccagtgcgttatatgacaacagcagtcaatgtcacccattctgggacagaaattgttgacttaatgtgccatgccaccttcacttcacgtctactacaaccaatcagagtccccaactataatctgtatattatggacgaggcccacttcacagatccctcaagtatagcagcaagaggatacatttcaacaagggttgagatgggcgaggcggccgccatcttcatgaccgccaccccaccaggaacccgtgacgcattcccggactccaactcaccaattatggacaccgaagtggaagtcccagagagagcctggagctcaggctttgattgggtgacggatcattctggaaaaacagtttggtttgttccaagcgtgaggaacggcaatgagatcgcagcttgtctgacaaaggctggaaaacgggtcatacagctcagcagaaagacttttgagacagagttcctgaaaacaaaaaatcaagagtgggacttcgtcgtgacaactgacatttcagagatgggcgccaactttaaagctgaccgtgtcatagattccaggagatgcctaaagccggtcatacttgatggcgagagagtcattctggctggacccatgcctgtcacacatgccagcgctgcccagaggagggggcgcataggcaggaatcccaacaaacctggagatgagtatctgtatggaggtgggtgcgcagagactgatgaagaccatgcacactggcttgaagcaagaatgcttcttgacaacatttacctccaagatggcctcatagcctcgctctatcgacctgaggccgacaaagtagcagctattgagggagagttcaagcttaggacggagcaaaggaagacctttgtggaactcatgaaaagaggagatcttcctgtttggctggcctatcaggttgcatctgccggaataacctacacagatagaaaatggtgctttgatggcacgaccaacaacaccataatggaagacagtgtgccggcagaggtgtggaccagatacggagagaaaagagtgctcaaaccaaggtggatggacgccagagtttgttcagatcatgcggccctgaagtcattcaaagagtttgccgctgggaaaagaggagyggcctttggagtgatggaagccctgggaacattgccgggacacatgacagagagattccaggaagccattgacaacctcgctgtgctcatgcgggcagagactggaagcaggccttacgaagccgcggcggcccaattgccggagaccttagagaccatcatgcttttggggttgctgggaacagtctcgctgggaatctttttcgtcttgatgcggaataagggcatcgggaagatgggctttggaatggtgactcttggggccagcgcatggcttatgtggctctcggaaattgagccagccagaattgcatgtgtcctcattgttgtgttcctattgctggtggtgctcatacctgagccagaaaagcaaagatctccccaggacaaccaaatggcaatcatcatcatgatagcagtgggtcttctgggtttgattaccgccaatgaacttggatggttggaaagaacaaagagtgacctaagccatctaatgggaaggagagaggagggggcaaccataggattctcaatggacattgacctgcggccagcctcagcttgggctatctatgctgctctgacaactttcatcaccccagccgtccaacatgcggtgaccacttcatacaacaactactccttaatggcgatggccacgcaagctggagtgttgtttggtatgggtaaagggatgccattctacgcatgggactttggagtcccgctgctaatgatgggttgctactcacaattaacacccctgaccctaatagtggccatcattttgctcgtggcgcactacatgtacttgatcccagggctgcaggcagcagctgcgcgtgctgcccagaagagaacggcagctggcatcatgaagaaccctgttgtggatggaatagtggtgactgacattgacacaatgacaattgaccaccgagtggagaaaaagatgggacaggtgctactcatagcagtagccgtctccagcgccatactgtcgcggaccgcctgggggtggggggaggctggggccctgatcacagctgcaacttccactttgtgggaaggctctccgaacaagtactggaactcctccacagccacttcactgtgtaacatttttaggggaagttacttggctggagcttctctaatctacacagtaacaagaaacgctggcttggtcaagagacgtgggggtggaacgggagagaccctgggagagaaatggaaggcccgcctgaaccagatgtcggccctagagttctactcctacaaaaagtcaggcatcaccgaggtgtgcagagaagaggcccgccgcgccctcaaggacggtgtggcaacaggaggccatgctgtgtcccgaggaagtgcaaagcttagatggttggtggagagaggatacctgcagccctatggaaaggtcattgatcttggatgtggcagagggggctggagttactacgccgccaccatccgcaaagttcaagaagtgaaaggatacacaaaaggaggccctggtcatgaagaacccatgttggtgcaaagctatgggtggaacatagtccgtcttaagagtggggtggacgtctttcatatggcggctgagccgtgtgacactttgctgtgtgatataggtgagtcatcatctagtcctgaagtggaagaagcacggacgctcagagtcctttccatggtgggggattggcttgaaaaaagaccaggagccttttgtataaaagtgttgtgcccatacaccagcactatgatggaaaccctggagcgactgcagcgtaggtatgggggaggactggtcagagtgccactctcccgcaactctacacatgagatgtactgggtctctggagcgaaaagcaacaccataaaaagtgtgtccaccacgagccagctcctcttggggcgcatggacgggcccaggaggccagtgaaatatgaggaggatgtgaatctcggctccggcacgcgggctgtggtaagctgcgctgaagctcccaacatgaagatcattggtaaccgcattgagaggatccgcagtgagcacgcggaaacgtggttctttgacgagaaccacccatataggacatgggcttaccatggaagctatgaggcccctacacaagggtcagcgtcctctctaataaacggggttgtcaggctcctgtcaaaaccctgggatgtggtgactggagtcacaggaatagccatgaccgacaccacaccgtatggtcagcaaagagttttcaaggaaaaagtggacactagggtgccagacccccaagaaggcactcgtcaggttatgagcatggtctcttcctggttatggaaagagctaggcaaacacaaacggccacgagtctgtaccaaagaagagttcatcaacaaggttcgtagcaatgcagcattaggggcaatatttgaagaggaaaaagagtggaagactgcagtggaagctgtgaacgatccaaggttctgggctctagtggacaaggaaagagagcaccacctgagaggagagtgtcagagctgtgtgtacaacatgatgggaaaaagagaaaagaaacaaggggaatttggaaaggccaagggcagccgcgccatctggtatatgtggctaggggctagattcctggagttcgaagcccttggattcttgaacgaggatcactggatggggagagagaattcaggaggtggtgttgaagggctgggattacaaagactcggatatgtcctagaagagatgagtcgcataccaggaggaaggatgtatgctgatgacacagctggctgggacacccgcatcagcaggtttgatctggagaatgaagctctaatcaccaaccaaatggagaaagggcacagggccttggcattggccataatcaagtacacataccaaaacaaagtggtaaaggtcctcagaccagctgaaaaagggaagacagttatggacattatttcaagacaagaccaaagggggagcggacaagttgtcacttacgctcttaatacattcaccaacctggtggtgcagctcattcggaatatggaggctgaggaagttctagagatgcaagacttgtggctgctgcggaggtcagagaaagtgaccaactggttgcagagcaacggatgggataggctcaaacgaatggcagtcagtggagatgattgcgttgtgaaaccaattgatgataggtttgcacatgccctcaggttcttgaatgatatgggaaaagtcaggaaggacacacaagagtggaaaccctcaactggatgggacaattgggaagaagttccgttttgctcccaccacttcaacaagctccatctcaaggacgggaggtccattgtggttccctgccgccaccaagatgaactgattggccgagcccgcgtctcaccaggggcgggatggagcatccgggagactgcttgcctagcaaaatcatatgcgcaaatgtggcagctcctttatttccacagaagggacctccgactgatggccaatgccatttgttcatctgtgccagttgactgggttccaactgggagaactacctggtcaatccatggaaagggagaatggatgaccactgaagacatgcttgtggtgtggaacagagtgtggattgaggagaacgaccacatggaagacaagaccccagttacgaaatggacagacattccctatttgggaaaaagggaagacttgtggtgtggatctctcatagggcacagaccgcgcactacctgggctgagaacatcaaaaacacagtcaacatgatgcgcaggatcataggtgatgaagaaaagtacatggactacctatccacccaagttcgctacttgggtgaagaagggtccacacccggagtgttgtaa

SEQ ID NO: 16 - protein, 8 aa, Artificial Sequence
  Description of Artificial Sequence: Synthetic 8xHis tag
HHHHHHHH